European Patent Application EP 4 306 641 A1, published January 17, 2024. Title: NOVEL NUCLEIC ACID MOLECULE. Applicant: ST Pharm Co., Ltd. The sequence listing filed with the application follows.

SEQUENCE LISTING (59 sequences)

SEQ ID NO: 1 - protein, 18 aa, Homo sapiens
MDWTWILFLVAAATRVHS

SEQ ID NO: 2 - RNA, 54 nt, Homo sapiens
atggactggacctggatcctcttcttggtggcagcagccacgcgagtccactcc

SEQ ID NO: 3 - RNA, 54 nt, Artificial Sequence
  IgE SP
atggactggacctggatcctgttcctggtggccgccgctacaagagtgcacagc

SEQ ID NO: 4 - RNA, 54 nt, Artificial Sequence
  IgE SP
atggactggacttggatcttgttcttggttgctgctgccaccagagtccactct

SEQ ID NO: 5 - protein, 18 aa, Homo sapiens
MKWVTFISLLFLFSSAYS

SEQ ID NO: 6 - RNA, 54 nt, Homo sapiens
atgaagtgggtaacctttatttcccttctttttctctttagctcggcttattcc

SEQ ID NO: 7 - RNA, 54 nt, Artificial Sequence
  albumin SP
atgaagtgggtgaccttcatcagcctgctgttcctgttttcttccgcctacagc

SEQ ID NO: 8 - RNA, 54 nt, Artificial Sequence
  albumin SP
atgaagtgggttactttcatctctttgttgtttttattctcctctgcttactcc

SEQ ID NO: 9 - protein, 23 aa, Homo sapiens
MKYTSYILAFQLCIVLGSLGCYC

SEQ ID NO: 10 - RNA, 69 nt, Homo sapiens
atgaaatatacaagttatatcttggcttttcagctctgcatcgttttgggttctcttggctgttactgc

SEQ ID NO: 11 - RNA, 69 nt, Artificial Sequence
  IFN-r SP
atgaagtacaccagctacatcctggccttccagctgtgcatcgtgctgggctctctgggctgttactgc

SEQ ID NO: 12 - RNA, 69 nt, Artificial Sequence
  IFN-r SP
atgaagtacacttcttacattttggctttccaattgtgtatcgttttgggttccttaggttgttactgt

SEQ ID NO: 13 - protein, 28 aa, Homo sapiens
MQRVNMIMAESPGLITICLLGYLLSAEC

SEQ ID NO: 14 - RNA, 84 nt, Homo sapiens
atgcagcgcgtgaacatgatcatggcagaatcaccaggcctcatcaccatctgccttttaggatatctactcagtgctgaatgt

SEQ ID NO: 15 - RNA, 84 nt, Artificial Sequence
  F IX
atgcagagagtgaacatgatcatggccgagtctcctggcctgatcaccatctgcctgctgggctacctgctgagcgccgaatgt

SEQ ID NO: 16 - RNA, 84 nt, Artificial Sequence
  F IX
atgcaaagagttaacatgattatggctgaatctccaggtttgatcactatctgtttgttgggttacttgttatccgccgaatgt

SEQ ID NO: 17 - protein, 20 aa, Homo sapiens
MVYKTLFALCILTAGWRVQS

SEQ ID NO: 18 - RNA, 60 nt, Homo sapiens
atggtctacaagactctcttcgctctttgcatcttaactgcaggatggagggtacagagt

SEQ ID NO: 19 - RNA, 60 nt, Artificial Sequence
  MLP1
atggtgtacaagaccctgttcgccctgtgcatcctgaccgccggctggagggtgcagagc

SEQ ID NO: 20 - RNA, 60 nt, Artificial Sequence
  MLP1
atggtatataaaactttatttgctttatgtattttaactgctggttggcgtgtacaatct

SEQ ID NO: 21 - protein, 1273 aa, Unknown
  SARS-CoV-2
MFVFLVLLPLVSSQCVNLTTRTQLPPAYTNSFTRGVYYPDKVFRSSVLHSTQDLFLPFFSNVTWFHAIHVSGTNGTKRFDNPVLPFNDGVYFASTEKSNIIRGWIFGTTLDSKTQSLLIVNNATNVVIKVCEFQFCNDPFLGVYYHKNNKSWMESEFRVYSSANNCTFEYVSQPFLMDLEGKQGNFKNLREFVFKNIDGYFKIYSKHTPINLVRDLPQGFSALEPLVDLPIGINITRFQTLLALHRSYLTPGDSSSGWTAGAAAYYVGYLQPRTFLLKYNENGTITDAVDCALDPLSETKCTLKSFTVEKGIYQTSNFRVQPTESIVRFPNITNLCPFGEVFNATRFASVYAWNRKRISNCVADYSVLYNSASFSTFKCYGVSPTKLNDLCFTNVYADSFVIRGDEVRQIAPGQTGKIADYNYKLPDDFTGCVIAWNSNNLDSKVGGNYNYLYRLFRKSNLKPFERDISTEIYQAGSTPCNGVEGFNCYFPLQSYGFQPTNGVGYQPYRVVVLSFELLHAPATVCGPKKSTNLVKNKCVNFNFNGLTGTGVLTESNKKFLPFQQFGRDIADTTDAVRDPQTLEILDITPCSFGGVSVITPGTNTSNQVAVLYQDVNCTEVPVAIHADQLTPTWRVYSTGSNVFQTRAGCLIGAEHVNNSYECDIPIGAGICASYQTQTNSPRRARSVASQSIIAYTMSLGAENSVAYSNNSIAIPTNFTISVTTEILPVSMTKTSVDCTMYICGDSTECSNLLLQYGSFCTQLNRALTGIAVEQDKNTQEVFAQVKQIYKTPPIKDFGGFNFSQILPDPSKPSKRSFIEDLLFNKVTLADAGFIKQYGDCLGDIAARDLICAQKFNGLTVLPPLLTDEMIAQYTSALLAGTITSGWTFGAGAALQIPFAMQMAYRFNGIGVTQNVLYENQKLIANQFNSAIGKIQDSLSSTASALGKLQDVVNQNAQALNTLVKQLSSNFGAISSVLNDILSRLDKVEAEVQIDRLITGRLQSLQTYVTQQLIRAAEIRASANLAATKMSECVLGQSKRVDFCGKGYHLMSFPQSAPHGVVFLHVTYVPAQEKNFTTAPAICHDGKAHFPREGVFVSNGTHWFVTQRNFYEPQIITTDNTFVSGNCDVVIGIVNNTVYDPLQPELDSFKEELDKYFKNHTSPDVDLGDISGINASVVNIQKEIDRLNEVAKNLNESLIDLQELGKYEQYIKWPWYIWLGFIAGLIAIVMVTIMLCCMTSCCSCLKGCCSCGSCCKFDEDDSEPVLKGVKLHYT

SEQ ID NO: 22 - RNA, 3822 nt, Unknown
  SARS-CoV-2
atgtttgtttttcttgttttattgccactagtctctagtcagtgtgttaatcttacaaccagaactcaattaccccctgcatacactaattctttcacacgtggtgtttattaccctgacaaagttttcagatcctcagttttacattcaactcaggacttgttcttacctttcttttccaatgttacttggttccatgctatacatgtctctgggaccaatggtactaagaggtttgataaccctgtcctaccatttaatgatggtgtttattttgcttccactgagaagtctaacataataagaggctggatttttggtactactttagattcgaagacccagtccctacttattgttaataacgctactaatgttgttattaaagtctgtgaatttcaattttgtaatgatccatttttgggtgtttattaccacaaaaacaacaaaagttggatggaaagtgagttcagagtttattctagtgcgaataattgcacttttgaatatgtctctcagccttttcttatggaccttgaaggaaaacagggtaatttcaaaaatcttagggaatttgtgtttaagaatattgatggttattttaaaatatattctaagcacacgcctattaatttagtgcgtgatctccctcagggtttttcggctttagaaccattggtagatttgccaataggtattaacatcactaggtttcaaactttacttgctttacatagaagttatttgactcctggtgattcttcttcaggttggacagctggtgctgcagcttattatgtgggttatcttcaacctaggacttttctattaaaatataatgaaaatggaaccattacagatgctgtagactgtgcacttgaccctctctcagaaacaaagtgtacgttgaaatccttcactgtagaaaaaggaatctatcaaacttctaactttagagtccaaccaacagaatctattgttagatttcctaatattacaaacttgtgcccttttggtgaagtttttaacgccaccagatttgcatctgtttatgcttggaacaggaagagaatcagcaactgtgttgctgattattctgtcctatataattccgcatcattttccacttttaagtgttatggagtgtctcctactaaattaaatgatctctgctttactaatgtctatgcagattcatttgtaattagaggtgatgaagtcagacaaatcgctccagggcaaactggaaagattgctgattataattataaattaccagatgattttacaggctgcgttatagcttggaattctaacaatcttgattctaaggttggtggtaattataattacctgtatagattgtttaggaagtctaatctcaaaccttttgagagagatatttcaactgaaatctatcaggccggtagcacaccttgtaatggtgttgaaggttttaattgttactttcctttacaatcatatggtttccaacccactaatggtgttggttaccaaccatacagagtagtagtactttcttttgaacttctacatgcaccagcaactgtttgtggacctaaaaagtctactaatttggttaaaaacaaatgtgtcaatttcaacttcaatggtttaacaggcacaggtgttcttactgagtctaacaaaaagtttctgcctttccaacaatttggcagagacattgctgacactactgatgctgtccgtgatccacagacacttgagattcttgacattacaccatgttcttttggtggtgtcagtgttataacaccaggaacaaatacttctaaccaggttgctgttctttatcaggatgttaactgcacagaagtccctgttgctattcatgcagatcaacttactcctacttggcgtgtttattctacaggttctaatgtttttcaaacacgtgcaggctgtttaataggggctgaacatgtcaacaactcatatgagtgtgacatacccattggtgcaggtatatgcgctagttatcagactcagactaattctcctcggcgggcacgtagtgtagctagtcaatccatcattgcctacactatgtcacttggtgcagaaaattcagttgcttactctaataactctattgccatacccacaaattttactattagtgttaccacagaaattctaccagtgtctatgaccaagacatcagtagattgtacaatgtacatttgtggtgattcaactgaatgcagcaatcttttgttgcaatatggcagtttttgtacacaattaaaccgtgctttaactggaatagctgttgaacaagacaaaaacacccaagaagtttttgcacaagtcaaacaaatttacaaaacaccaccaattaaagattttggtggttttaatttttcacaaatattaccagatccatcaaaaccaagcaagaggtcatttattgaagatctacttttcaacaaagtgacacttgcagatgctggcttcatcaaacaatatggtgattgccttggtgatattgctgctagagacctcatttgtgcacaaaagtttaacggccttactgttttgccacctttgctcacagatgaaatgattgctcaatacacttctgcactgttagcgggtacaatcacttctggttggacctttggtgcaggtgctgcattacaaataccatttgctatgcaaatggcttataggtttaatggtattggagttacacagaatgttctctatgagaaccaaaaattgattgccaaccaatttaatagtgctattggcaaaattcaagactcactttcttccacagcaagtgcacttggaaaacttcaagatgtggtcaaccaaaatgcacaagctttaaacacgcttgttaaacaacttagctccaattttggtgcaatttcaagtgttttaaatgatatcctttcacgtcttgacaaagttgaggctgaagtgcaaattgataggttgatcacaggcagacttcaaagtttgcagacatatgtgactcaacaattaattagagctgcagaaatcagagcttctgctaatcttgctgctactaaaatgtcagagtgtgtacttggacaatcaaaaagagttgatttttgtggaaagggctatcatcttatgtccttccctcagtcagcacctcatggtgtagtcttcttgcatgtgacttatgtccctgcacaagaaaagaacttcacaactgctcctgccatttgtcatgatggaaaagcacactttcctcgtgaaggtgtctttgtttcaaatggcacacactggtttgtaacacaaaggaatttttatgaaccacaaatcattactacagacaacacatttgtgtctggtaactgtgatgttgtaataggaattgtcaacaacacagtttatgatcctttgcaacctgaattagactcattcaaggaggagttagataaatattttaagaatcatacatcaccagatgttgatttaggtgacatctctggcattaatgcttcagttgtaaacattcaaaaagaaattgaccgcctcaatgaggttgccaagaatttaaatgaatctctcatcgatctccaagaacttggaaagtatgagcagtatataaaatggccatggtacatttggctaggttttatagctggcttgattgccatagtaatggtgacaattatgctttgctgtatgaccagttgctgtagttgtctcaagggctgttgttcttgtggatcctgctgcaaatttgatgaagacgactctgagccagtgctcaaaggagtcaaattacattacacataa

SEQ ID NO: 23 - RNA, 3822 nt, Artificial Sequence
  SARS-CoV-2 S
atgttcgtgttcttggtgctgctgcctctggtctccagccagtgcgtgaatctgaccaccagaacccaactgcctcctgcctacaccaacagcttcacaagaggcgtgtactaccccgacaaggtgttccggagtagcgtgctgcacagcacgcaggacctgttcctgccatttttctctaatgtgacctggtttcacgccatccacgtgtccggcacaaacggcacaaagcggttcgacaaccccgtgctgccattcaacgatggcgtgtacttcgcctctacagaaaagtccaatatcattaggggctggatcttcggaacaacgctggactcaaagacccagagcctgctgatcgtcaataacgccacaaatgtggtcattaaagtgtgcgaattccagttctgcaacgaccccttcctgggcgtctactatcataagaacaacaagtcttggatggaaagcgagttccgggtgtacagcagcgctaacaactgcaccttcgagtacgtttcccaacctttcctgatggacctggaaggcaagcagggcaatttcaagaacctgagagaattcgtgttcaagaacatcgacggctacttcaagatctacagcaagcacacccccatcaacctggtacgagatctgccccagggcttctctgccctcgagcccctcgtggacctgcccattggaatcaacatcacgcggttccagaccctgctcgccctgcatagaagctacctcactcccggcgattctagcagcggctggacagccggcgctgccgcttactacgtgggctacctgcagcctagaacatttctactgaagtataacgagaacgggacaatcacagacgccgtggactgcgctctggatcctctgagcgaaaccaagtgcaccctgaaaagcttcaccgtcgagaagggaatctaccagacctccaacttccgggtgcagccaaccgagagcatcgtgagattccctaacatcactaacctgtgtccttttggagaagtgttcaacgccacccggttcgccagcgtttatgcctggaaccgcaagagaatctctaactgtgtggccgactacagcgtgctgtacaattctgccagcttcagcaccttcaagtgctacggcgtgagtcccaccaaactgaacgacctgtgcttcactaacgtgtacgccgatagctttgtgatcagaggagacgaggtgagacagattgctcctggccagaccggcaaaatcgccgattacaactacaagctacctgacgacttcaccggctgcgtgatcgcctggaattctaacaacctggactccaaggtgggcggcaactacaactacctgtacagactgtttcggaagtccaacctgaaaccattcgagagagatatcagcacagagatctaccaagcgggctcgacaccttgcaacggagtggagggcttcaactgttactttcctctgcagtcttatggcttccaacctacaaatggcgtcggatatcagccctacagagtggtggtgctttctttcgagctgctgcacgccccagctaccgtgtgtggtcctaagaagtcgacaaatctggtgaagaataagtgcgtgaattttaactttaacggcctgaccggcaccggcgtgctgaccgaatctaacaagaaattcctgcctttccagcagttcggtagagatatcgccgacaccaccgatgccgtgcgggaccctcaaacactggaaatcctggacataacaccttgcagcttcggcggagtcagcgtgatcacacctggcaccaacaccagcaaccaggtggccgtgctgtaccaggacgtgaactgcacagaagtgcctgtggcgatccacgctgatcagctgacacctacatggcgggtgtactcaacaggaagcaacgtgtttcagacccgggccggctgtctgatcggcgctgaacacgttaacaacagctacgagtgcgacatccccatcggcgccggcatctgtgccagctaccagactcagacaaatagccctaggagagcaagatccgtggccagccagagcatcatcgcctatacaatgagcctgggcgccgagaattctgtcgcctacagcaacaacagcatcgccatccccactaatttcaccatctccgtcaccacagaaatcctgcctgtgagcatgaccaagaccagcgtggattgcacaatgtacatttgcggcgacagcaccgagtgttccaacctgctgctgcagtacggcagcttctgcacccagctgaacagagcactgacaggcatcgccgtggagcaagacaagaacacccaggaggtgttcgcccaggtgaagcagatctacaagacccctcctatcaaagacttcggtggcttcaacttcagccagatcctgcctgatccgagcaagcctagcaaaagatcatttatcgaagacctgctgtttaacaaggtgaccctggccgacgccggattcatcaagcagtacggcgactgcctgggcgacatcgccgccagagatctgatctgtgcccagaagtttaatggcctgaccgtgctgccacctctgctgaccgacgagatgatcgcccaatataccagcgccctgctggctggaacaatcacaagcggctggaccttcggagccggagccgctcttcagattcctttcgccatgcagatggcctacagattcaacggcatcggcgtgacccagaacgtgctgtatgagaaccagaaactgatcgctaatcaatttaacagcgccatcggcaagattcaggactccctgagctcaacagcctctgccctgggcaagctgcaggatgtggtgaaccagaacgcccaggccctgaacacactggtgaaacagctgtcaagcaacttcggcgccatctcatccgtactgaacgacatcctgtctagactcgataaggtggaggccgaagtgcagatcgacagactgatcaccggccggctgcagagcctgcagacgtacgtgacccaacagctgatcagggccgccgagatccgggcctcggctaatttggccgccaccaaaatgagcgaatgcgtgctgggccagtctaagagggtcgacttctgtggcaagggctaccacctgatgagcttcccccagagcgctccccacggcgtggtgttcctgcacgtgacctacgttccagcccaggagaagaactttacaaccgcccctgccatctgccacgacggcaaggcccacttccctagagagggagtctttgtgagcaatggcacccactggttcgttacccagagaaacttctacgagccccagatcatcaccacagacaacaccttcgtgagcggaaactgtgacgtggtgatcggcatcgtgaacaacaccgtgtacgaccccctgcaacccgagctggacagcttcaaggaagagctggacaaatactttaagaaccacacctcacctgacgtggacctgggagatatcagcggcataaatgcctccgtggtgaacatccagaaggaaatcgatagactcaatgaggtggctaagaacctgaacgaaagcctgatcgacctccaagagctgggcaaatacgagcagtacatcaagtggccttggtacatttggctgggctttatcgccggcctcatcgctatcgtgatggtgaccatcatgctgtgctgcatgacctcctgctgcagctgcctgaagggctgttgcagctgcggcagctgctgcaagttcgacgaagatgattctgaaccagtgctgaaaggcgtgaaactgcactacacctga

SEQ ID NO: 24 - RNA, 3822 nt, Artificial Sequence
  SARS-CoV-2 S
atgttcgtgttcctcgtcttgctacctttggtttcttctcaatgtgttaatttgactaccagaacccaattaccaccagcttacaccaattcttttaccagaggtgtctattacccagacaaggtcttcagatcttctgtattgcactctactcaagacttgttcttaccattcttctccaacgttacctggtttcacgctatccatgttagtggtaccaacggtaccaagagattcgacaacccagttttacctttcaacgatggtgtttactttgcttcaaccgaaaagtctaacatcatcagaggttggattttcggtaccactttggattcaaaaactcaatctttgttgattgttaacaatgccactaatgttgttatcaaggtttgtgaattccaattttgtaacgacccattcttgggtgtctactaccacaagaacaacaagtcttggatggagtctgaattcagagtttactcttctgctaacaactgtactttcgaatacgtttctcaaccatttttgatggacttggaaggtaaacaaggtaacttcaaaaacttgagagaattcgtcttcaaaaacattgacggttacttcaagatctactctaagcacaccccaatcaacctagtaagagatttgccacaaggtttctccgccctagaaccattggttgatttgccaattggtattaacatcaccagattccaaaccttgttggctttgcacagatcctacttgactccaggtgattcttcttccggttggaccgctggtgccgctgcatactacgtcggttacttgcaaccaagaactttcttgttgaagtacaacgaaaatggtactatcactgatgctgtcgattgcgctttggacccattgtctgaaaccaagtgtactttgaagtcttttactgttgaaaagggtatctaccaaacttctaacttcagagtccaaccaaccgaatctatcgtccgattcccaaacattactaacttatgtccattcggtgaagttttcaacgctaccagattcgcttccgtctacgcttggaacagaaagagaatctcgaattgtgttgccgactactccgttttgtacaactccgcttccttttccaccttcaagtgttacggtgtttctccaactaagctaaacgatttgtgtttcaccaacgtctacgccgactccttcgttattagaggtgacgaggtcagacaaattgctccaggtcaaaccgggaaaatcgctgattacaactacaaattaccagatgacttcactggttgtgtcatcgcttggaactccaacaacttggattctaaagttggtggtaattataactatttatacagattattcagaaagtcaaacttgaaaccatttgaaagagacatctccactgaaatttatcaagctggttctactccatgtaacggtgtcgaaggtttcaactgttatttcccattgcaatcctacggtttccagccaacaaacggtgtcggttaccaaccgtacagagtcgttgtcctttcctttgaattgttgcacgctcctgccactgtctgtggtccaaagaagtccaccaacttggtcaaaaacaagtgtgtgaacttcaactttaacggtttgactggaacaggtgttttgactgaatccaacaagaagttcttgcctttccaacaatttggtagagacattgccgatactactgatgccgtcagagaccctcaaactttggaaatcttggatataactccatgctccttcggtggagtctctgtcataactccaggtaccaacacctcgaaccaagttgctgttttgtaccaagatgtcaactgtactgaagttccggtcgccatccatgctgatcaattgacaccaacttggcgtgtttactctaccggctctaacgtctttcaaaccagagctggttgtttgattggtgctgaacacgttaacaactcttatgaatgtgatattccaatcggtgccggtatctgtgcttcctaccaaacgcaaaccaactctccacgtagagctcgtagtgttgcatcacaatctattatcgcctacactatgtctcttggtgctgaaaattctgttgcctacagtaacaactctatcgccatcccaaccaactttaccatctccgttactaccgaaattctgccagtctccatgaccaagacttccgttgattgcaccatgtacatatgtggtgactccactgaatgttccaacttgttgttgcaatacggttccttctgtactcaattaaacagagcattgaccggtatcgctgtcgaacaagataaaaacacccaagaagtgttcgctcaagttaagcaaatctacaagaccccaccaatcaaggacttcggaggtttcaacttctctcaaatcttgccagacccatctaagccatccaagcgttctttcattgaagacttgttgttcaacaaggttaccttggctgatgcaggtttcatcaagcaatacggtgactgtttgggtgacatcgctgccagggatctgatctgtgcccaaaagttcaacggtttaactgttttgccacctttattaaccgatgaaatgattgctcaatacacctcggctttgttggctggtaccatcacgtctggttggactttcggtgctggtgctgctcttcaaatcccttttgctatgcaaatggcttacagatttaacggtattggtgttacgcaaaacgttttgtacgaaaaccaaaagttgatcgctaaccaattcaactctgctattggtaagatccaagactccttgagttcgaccgcgtctgctttgggtaagttgcaagatgttgttaaccaaaacgcccaagctctcaacactttggtcaagcaactttcttccaacttcggtgctatctcttctgttctgaacgacattttgtccagactagataaggttgaagctgaagttcaaatcgacagattgatcaccggtagattgcaaagcctacaaacttacgtaacccaacaattaataagagctgccgaaattcgtgcttctgccaacttggctgctaccaagatgtccgaatgtgttttgggtcaatctaagcgtgtcgatttctgtggtaaaggttaccatttgatgtctttcccacaatccgctccacacggtgttgtcttcttgcatgttacctacgtcccagctcaagaaaagaacttcactactgctccagctatctgtcacgatggtaaggctcacttcccaagagaaggtgttttcgtttctaatgggactcactggttcgttactcaaagaaacttctacgaaccacaaattattactactgacaacacttttgtttccggtaactgtgacgtcgtgattggtattgtcaacaataccgtctacgatcctctacagccagaattggattcatttaaggaagaattggacaagtacttcaagaatcacacttctccagacgtcgacttgggtgacatttctggtatcaacgcttctgttgtcaacattcaaaaggaaatcgacagattgaacgaagtcgctaagaacttgaacgaatcattaattgacttgcaagaattaggtaagtacgaacaatacattaaatggccatggtatatctggttgggttttatcgctggtctaattgccattgttatggttactattatgttatgttgtatgacttcttgctgctcttgtttgaaggggtgttgtagctgcggttcttgttgtaagttcgatgaagacgactctgaaccagttttaaagggtgtcaagctccactacacttga

SEQ ID NO: 25 - RNA, 3822 nt, Artificial Sequence
  SARS-CoV-2 S
atgttcgtgttcctcgtcttgctacctttggtttcttctcaatgtgttaatttgactaccagaacccaattaccaccagcttacaccaattcttttaccagaggcgtgtactaccccgacaaggtgttccggagtagcgtgctgcacagcacgcaggacctgttcctgccatttttctctaatgtgacctggtttcacgccatccacgtgtccggcacaaacggcacaaagcggttcgacaaccccgtgctgccattcaacgatggcgtgtacttcgcctctacagaaaagtccaatatcattaggggctggatcttcggaacaacgctggactcaaagacccagagcctgctgatcgtcaataacgccacaaatgtggtcattaaagtgtgcgaattccagttctgcaacgaccccttcctgggcgtctactatcataagaacaacaagtcttggatggaaagcgagttccgggtgtacagcagcgctaacaactgcaccttcgagtacgtttcccaacctttcctgatggacctggaaggcaagcagggcaatttcaagaacctgagagaattcgtgttcaagaacatcgacggctacttcaagatctacagcaagcacacccccatcaacctggtacgagatctgccccagggcttctctgccctcgagcccctcgtggacctgcccattggaatcaacatcacgcggttccagaccctgctcgccctgcatagaagctacctcactcccggcgattctagcagcggctggacagccggcgctgccgcttactacgtgggctacctgcagcctagaacatttctactgaagtataacgagaacgggacaatcacagacgccgtggactgcgctctggatcctctgagcgaaaccaagtgcaccctgaaaagcttcaccgtcgagaagggaatctaccagacctccaacttccgggtgcagccaaccgagagcatcgtgagattccctaacatcactaacctgtgtccttttggagaagtgttcaacgccacccggttcgccagcgtttatgcctggaaccgcaagagaatctctaactgtgtggccgactacagcgtgctgtacaattctgccagcttcagcaccttcaagtgctacggcgtgagtcccaccaaactgaacgacctgtgcttcactaacgtgtacgccgatagctttgtgatcagaggagacgaggtgagacagattgctcctggccagaccggcaaaatcgccgattacaactacaagctacctgacgacttcaccggctgcgtgatcgcctggaattctaacaacctggactccaaggtgggcggcaactacaactacctgtacagactgtttcggaagtccaacctgaaaccattcgagagagatatcagcacagagatctaccaagcgggctcgacaccttgcaacggagtggagggcttcaactgttactttcctctgcagtcttatggcttccaacctacaaatggcgtcggatatcagccctacagagtggtggtgctttctttcgagctgctgcacgccccagctaccgtgtgtggtcctaagaagtcgacaaatctggtgaagaataagtgcgtgaattttaactttaacggcctgaccggcaccggcgtgctgaccgaatctaacaagaaattcctgcctttccagcagttcggtagagatatcgccgacaccaccgatgccgtgcgggaccctcaaacactggaaatcctggacataacaccttgcagcttcggcggagtcagcgtgatcacacctggcaccaacaccagcaaccaggtggccgtgctgtaccaggacgtgaactgcacagaagtgcctgtggcgatccacgctgatcagctgacacctacatggcgggtgtactcaacaggaagcaacgtgtttcagacacgggccggctgtctgatcggcgctgaacacgttaacaacagctacgagtgcgacatccccatcggcgccggcatctgtgccagctaccagactcagacaaatagccctaggagagcaagatccgtggccagccagagcatcatcgcctatacaatgagcctgggcgccgagaattctgtcgcctacagcaacaacagcatcgccatccccactaatttcaccatctccgtcaccacagaaatcctgcctgtgagcatgaccaagaccagcgtggattgcacaatgtacatttgcggcgacagcaccgagtgttccaacctgctgctgcagtacggcagcttctgcacccagctgaacagagcactgacaggcatcgccgtggagcaagacaagaacacccaggaggtgttcgcccaggtgaagcagatctacaagacccctcctatcaaagacttcggtggcttcaacttcagccagatcctgcctgatccgagcaagcctagcaaaagatcatttatcgaagacctgctgtttaacaaggtgaccctggccgacgccggattcatcaagcagtacggcgactgcctgggcgacatcgccgccagagatctgatctgtgcccagaagtttaatggcctgaccgtgctgccacctctgctgaccgacgagatgatcgcccaatataccagcgccctgctggctggaacaatcacaagcggctggaccttcggagccggagccgctcttcagattcctttcgccatgcagatggcctacagattcaacggcatcggcgtgacccagaacgtgctgtatgagaaccagaaactgatcgctaatcaatttaacagcgccatcggcaagattcaggactccctgagctcaacagcctctgccctgggcaagctgcaggatgtggtgaaccagaacgcccaggccctgaacacactggtgaaacagctgtcaagcaacttcggcgccatctcatccgtactgaacgacatcctgtctagactcgatccaccagaggccgaagtgcagatcgacagactgatcaccggccggctgcagagcctgcagacgtacgtgacccaacagctgatcagggccgccgagatccgggcctcggctaatttggccgccaccaaaatgagcgaatgcgtgctgggccagtctaagagggtcgacttctgtggcaagggctaccacctgatgagcttcccccagagcgctccccacggcgtggtgttcctgcacgtgacctacgttccagcccaggagaagaactttacaaccgcccctgccatctgccacgacggcaaggcccacttccctagagagggagtctttgtgagcaatggcacccactggttcgttacccagagaaacttctacgagccccagatcatcaccacagacaacaccttcgtgagcggaaactgtgacgtggtgatcggcatcgtgaacaacaccgtgtacgaccccctgcaacccgagctggacagcttcaaggaagagctggacaaatactttaagaaccacacctcacctgacgtggacctgggagatatcagcggcataaatgcctccgtggtgaacatccagaaggaaatcgatagactcaatgaggtggctaagaacctgaacgaaagcctgatcgacctccaagagctgggcaaatacgagcagtacatcaagtggccttggtacatttggctgggctttatcgccggcctcatcgctatcgtgatggtgaccatcatgctgtgctgcatgacctcctgctgcagctgcctgaagggctgttgcagctgcggcagctgctgcaagttcgacgaagatgattctgaaccagtgctgaaaggcgtgaaactgcactacacctga

SEQ ID NO: 26 - protein, 222 aa, Unknown
  SARS-CoV-2
MADSNGTITVEELKKLLEQWNLVIGFLFLTWICLLQFAYANRNRFLYIIKLIFLWLLWPVTLACFVLAAVYRINWITGGIAIAMACLVGLMWLSYFIASFRLFARTRSMWSFNPETNILLNVPLHGTILTRPLLESELVIGAVILRGHLRIAGHHLGRCDIKDLPKEITVATSRTLSYYKLGASQRVAGDSGFAAYSRYRIGNYKLNTDHSSSSDNIALLVQ

SEQ ID NO: 27 - RNA, 669 nt, Unknown
  SARS-CoV-2
atggcagattccaacggtactattaccgttgaagagcttaaaaagctccttgaacaatggaacctagtaataggtttcctattccttacatggatttgtcttctacaatttgcctatgccaacaggaataggtttttgtatataattaagttaattttcctctggctgttatggccagtaactttagcttgttttgtgcttgctgctgtttacagaataaattggatcaccggtggaattgctatcgcaatggcttgtcttgtaggcttgatgtggctcagctacttcattgcttctttcagactgtttgcgcgtacgcgttccatgtggtcattcaatccagaaactaacattcttctcaacgtgccactccatggcactattctgaccagaccgcttctagaaagtgaactcgtaatcggagctgtgatccttcgtggacatcttcgtattgctggacaccatctaggacgctgtgacatcaaggacctgcctaaagaaatcactgttgctacatcacgaacgctttcttattacaaattgggagcttcgcagcgtgtagcaggtgactcaggttttgctgcatacagtcgctacaggattggcaactataaattaaacacagaccattccagtagcagtgacaatattgctttgcttgtacagtaa

SEQ ID NO: 28 - RNA, 669 nt, Artificial Sequence
  SARS-CoV-2 M
atggctgatagcaacggcaccatcacagtcgaggaactgaaaaagctgctggaacagtggaacctggtgattggattcctgttcctgacctggatctgcctgctccagttcgcctacgccaaccggaacagattcctgtacatcatcaagctgatcttcctgtggctgctgtggcctgtgaccctggcctgcttcgtgctggctgctgtgtacagaatcaactggatcaccggaggcatcgccatcgccatggcctgtctggtgggcctgatgtggctgagctacttcatcgcctcttttagactgtttgccagaacccggagcatgtggtccttcaaccccgagacaaacatcctgctgaatgtgcccctgcacggcacaatcctgacaagacctctgcttgagagcgagctggtgatcggcgccgtgatcctgaggggccatctgcggattgccggacaccacctgggcagatgcgacatcaaggacctgcctaaggaaatcaccgtggctacaagccgcaccctgtcctactacaaactcggcgccagccaaagagtggccggcgacagcggcttcgccgcctatagcagataccggatcggcaactacaagctgaacaccgaccactctagcagctctgataatatcgccctgctggttcagtga

SEQ ID NO: 29 - RNA, 669 nt, Artificial Sequence
  SARS-CoV-2 M
atggctgattccaacggtaccatcaccgttgaagaattgaagaagttgctggaacaatggaacttggtcattggttttttattcttgacttggatctgtttgttgcaattcgcttacgctaacagaaaccgtttcctctacattatcaagttgatcttcctatggttattgtggccagtcactttggcttgtttcgttttggccgcagtttacagaatcaactggattacaggtggtattgctattgctatggcctgtttggttggtttgatgtggttgtcttacttcatcgcttccttcagattatttgctagaaccagatccatgtggtctttcaacccagaaaccaacatcttgttgaatgttccattgcacggtactatcttaaccagacctttattggaatctgaattagttatcggtgctgtcattttgcgtggtcacttgagaattgctggtcatcacttgggtagatgcgatatcaaggatttgccaaaggaaatcactgttgctaccagcagaactttgtcctactacaagttgggcgcttctcaaagagtcgccggtgactctggtttcgccgcctattcaagataccgtattggtaactacaaattgaacactgaccactcttcttcctctgacaacattgctttgttggtccaatga

SEQ ID NO: 30 - RNA, 669 nt, Artificial Sequence
  SARS-CoV-2 M
atggctgattccaacggtaccatcaccgttgaagaattgaagaagttgctggaacaatggaacttggtcattggttttttattcttgacttggatctgtttgttgcaattcgcttacgctaacagaaaccgtttcctctacattatcaagttgatcttcctatggttattgtggccagtcactttggcttgtttcgttttggccgcagtttacagaatcaactggattacaggtggtattgctattgctatggcctgtctggtgggcctgatgtggctgagctacttcatcgcctcttttagactgtttgccagaacccggagcatgtggtccttcaaccccgagacaaacatcctgctgaatgtgcccctgcacggcacaatcctgacaagacctctgcttgagagcgagctggtgatcggcgccgtgatcctgaggggccatctgcggattgccggacaccacctgggcagatgcgacatcaaggacctgcctaaggaaatcaccgtggctacaagccgcaccctgtcctactacaaactcggcgccagccaaagagtggccggcgacagcggcttcgccgcctatagcagataccggatcggcaactacaagctgaacaccgaccactctagcagctctgataatatcgccctgctggttcagtga

SEQ ID NO: 31 - RNA, 3873 nt, Artificial Sequence
  IgE SP - SARS-CoV-2 S
atggactggacttggatcttgttcttggttgctgctgccaccagagtccactctttcgtgttcctcgtcttgctacctttggtttcttctcaatgtgttaatttgactaccagaacccaattaccaccagcttacaccaattcttttaccagaggcgtgtactaccccgacaaggtgttccggagtagcgtgctgcacagcacgcaggacctgttcctgccatttttctctaatgtgacctggtttcacgccatccacgtgtccggcacaaacggcacaaagcggttcgacaaccccgtgctgccattcaacgatggcgtgtacttcgcctctacagaaaagtccaatatcattaggggctggatcttcggaacaacgctggactcaaagacccagagcctgctgatcgtcaataacgccacaaatgtggtcattaaagtgtgcgaattccagttctgcaacgaccccttcctgggcgtctactatcataagaacaacaagtcttggatggaaagcgagttccgggtgtacagcagcgctaacaactgcaccttcgagtacgtttcccaacctttcctgatggacctggaaggcaagcagggcaatttcaagaacctgagagaattcgtgttcaagaacatcgacggctacttcaagatctacagcaagcacacccccatcaacctggtacgagatctgccccagggcttctctgccctcgagcccctcgtggacctgcccattggaatcaacatcacgcggttccagaccctgctcgccctgcatagaagctacctcactcccggcgattctagcagcggctggacagccggcgctgccgcttactacgtgggctacctgcagcctagaacatttctactgaagtataacgagaacgggacaatcacagacgccgtggactgcgctctggatcctctgagcgaaaccaagtgcaccctgaaaagcttcaccgtcgagaagggaatctaccagacctccaacttccgggtgcagccaaccgagagcatcgtgagattccctaacatcactaacctgtgtccttttggagaagtgttcaacgccacccggttcgccagcgtttatgcctggaaccgcaagagaatctctaactgtgtggccgactacagcgtgctgtacaattctgccagcttcagcaccttcaagtgctacggcgtgagtcccaccaaactgaacgacctgtgcttcactaacgtgtacgccgatagctttgtgatcagaggagacgaggtgagacagattgctcctggccagaccggcaaaatcgccgattacaactacaagctacctgacgacttcaccggctgcgtgatcgcctggaattctaacaacctggactccaaggtgggcggcaactacaactacctgtacagactgtttcggaagtccaacctgaaaccattcgagagagatatcagcacagagatctaccaagcgggctcgacaccttgcaacggagtggagggcttcaactgttactttcctctgcagtcttatggcttccaacctacaaatggcgtcggatatcagccctacagagtggtggtgctttctttcgagctgctgcacgccccagctaccgtgtgtggtcctaagaagtcgacaaatctggtgaagaataagtgcgtgaattttaactttaacggcctgaccggcaccggcgtgctgaccgaatctaacaagaaattcctgcctttccagcagttcggtagagatatcgccgacaccaccgatgccgtgcgggaccctcaaacactggaaatcctggacataacaccttgcagcttcggcggagtcagcgtgatcacacctggcaccaacaccagcaaccaggtggccgtgctgtaccaggacgtgaactgcacagaagtgcctgtggcgatccacgctgatcagctgacacctacatggcgggtgtactcaacaggaagcaacgtgtttcagacccgggccggctgtctgatcggcgctgaacacgttaacaacagctacgagtgcgacatccccatcggcgccggcatctgtgccagctaccagactcagacaaatagccctaggagagcaagatccgtggccagccagagcatcatcgcctatacaatgagcctgggcgccgagaattctgtcgcctacagcaacaacagcatcgccatccccactaatttcaccatctccgtcaccacagaaatcctgcctgtgagcatgaccaagaccagcgtggattgcacaatgtacatttgcggcgacagcaccgagtgttccaacctgctgctgcagtacggcagcttctgcacccagctgaacagagcactgacaggcatcgccgtggagcaagacaagaacacccaggaggtgttcgcccaggtgaagcagatctacaagacccctcctatcaaagacttcggtggcttcaacttcagccagatcctgcctgatccgagcaagcctagcaaaagatcatttatcgaagacctgctgtttaacaaggtgaccctggccgacgccggattcatcaagcagtacggcgactgcctgggcgacatcgccgccagagatctgatctgtgcccagaagtttaatggcctgaccgtgctgccacctctgctgaccgacgagatgatcgcccaatataccagcgccctgctggctggaacaatcacaagcggctggaccttcggagccggagccgctcttcagattcctttcgccatgcagatggcctacagattcaacggcatcggcgtgacccagaacgtgctgtatgagaaccagaaactgatcgctaatcaatttaacagcgccatcggcaagattcaggactccctgagctcaacagcctctgccctgggcaagctgcaggatgtggtgaaccagaacgcccaggccctgaacacactggtgaaacagctgtcaagcaacttcggcgccatctcatccgtactgaacgacatcctgtctagactcgatccaccagaggccgaagtgcagatcgacagactgatcaccggccggctgcagagcctgcagacgtacgtgacccaacagctgatcagggccgccgagatccgggcctcggctaatttggccgccaccaaaatgagcgaatgcgtgctgggccagtctaagagggtcgacttctgtggcaagggctaccacctgatgagcttcccccagagcgctccccacggcgtggtgttcctgcacgtgacctacgttccagcccaggagaagaactttacaaccgcccctgccatctgccacgacggcaaggcccacttccctagagagggagtctttgtgagcaatggcacccactggttcgttacccagagaaacttctacgagccccagatcatcaccacagacaacaccttcgtgagcggaaactgtgacgtggtgatcggcatcgtgaacaacaccgtgtacgaccccctgcaacccgagctggacagcttcaaggaagagctggacaaatactttaagaaccacacctcacctgacgtggacctgggagatatcagcggcataaatgcctccgtggtgaacatccagaaggaaatcgatagactcaatgaggtggctaagaacctgaacgaaagcctgatcgacctccaagagctgggcaaatacgagcagtacatcaagtggccttggtacatttggctgggctttatcgccggcctcatcgctatcgtgatggtgaccatcatgctgtgctgcatgacctcctgctgcagctgcctgaagggctgttgcagctgcggcagctgctgcaagttcgacgaagatgattctgaaccagtgctgaaaggcgtgaaactgcactacacctga

SEQ ID NO: 32 - RNA, 4059 nt, Artificial Sequence
  albumin SP - SARS-CoV-2 S
atgaagtgggttactttcatctctttgttgtttttattctcctctgcttactccttcgtgttcctcgtcttgctacctttggtttcttctcaatgtgttaatttgactaccagaacccaattaccaccagcttacaccaattcttttaccagaggcgtgtactaccccgacaaggtgttccggagtagcgtgctgcacagcacgcaggacctgttcctgccatttttctctaatgtgacctggtttcacgccatccacgtgtccggcacaaacggcacaaagcggttcgacaaccccgtgctgccattcaacgatggcgtgtacttcgcctctacagaaaagtccaatatcattaggggctggatcttcggaacaacgctggactcaaagacccagaggattcttgacattacaccatgttcttttggtggtgtcagtgttataacaccaggaacaaatacttctaaccaggttgctgttctttatcaggatgttaactgcacagaagtccctgttgctattcatgcagatcaacttactcctacttggcgtgtttattctacaggttctaatgtttttcaaaccctgctgatcgtcaataacgccacaaatgtggtcattaaagtgtgcgaattccagttctgcaacgaccccttcctgggcgtctactatcataagaacaacaagtcttggatggaaagcgagttccgggtgtacagcagcgctaacaactgcaccttcgagtacgtttcccaacctttcctgatggacctggaaggcaagcagggcaatttcaagaacctgagagaattcgtgttcaagaacatcgacggctacttcaagatctacagcaagcacacccccatcaacctggtacgagatctgccccagggcttctctgccctcgagcccctcgtggacctgcccattggaatcaacatcacgcggttccagaccctgctcgccctgcatagaagctacctcactcccggcgattctagcagcggctggacagccggcgctgccgcttactacgtgggctacctgcagcctagaacatttctactgaagtataacgagaacgggacaatcacagacgccgtggactgcgctctggatcctctgagcgaaaccaagtgcaccctgaaaagcttcaccgtcgagaagggaatctaccagacctccaacttccgggtgcagccaaccgagagcatcgtgagattccctaacatcactaacctgtgtccttttggagaagtgttcaacgccacccggttcgccagcgtttatgcctggaaccgcaagagaatctctaactgtgtggccgactacagcgtgctgtacaattctgccagcttcagcaccttcaagtgctacggcgtgagtcccaccaaactgaacgacctgtgcttcactaacgtgtacgccgatagctttgtgatcagaggagacgaggtgagacagattgctcctggccagaccggcaaaatcgccgattacaactacaagctacctgacgacttcaccggctgcgtgatcgcctggaattctaacaacctggactccaaggtgggcggcaactacaactacctgtacagactgtttcggaagtccaacctgaaaccattcgagagagatatcagcacagagatctaccaagcgggctcgacaccttgcaacggagtggagggcttcaactgttactttcctctgcagtcttatggcttccaacctacaaatggcgtcggatatcagccctacagagtggtggtgctttctttcgagctgctgcacgccccagctaccgtgtgtggtcctaagaagtcgacaaatctggtgaagaataagtgcgtgaattttaactttaacggcctgaccggcaccggcgtgctgaccgaatctaacaagaaattcctgcctttccagcagttcggtagagatatcgccgacaccaccgatgccgtgcgggaccctcaaacactggaaatcctggacataacaccttgcagcttcggcggagtcagcgtgatcacacctggcaccaacaccagcaaccaggtggccgtgctgtaccaggacgtgaactgcacagaagtgcctgtggcgatccacgctgatcagctgacacctacatggcgggtgtactcaacaggaagcaacgtgtttcagacacgggccggctgtctgatcggcgctgaacacgttaacaacagctacgagtgcgacatccccatcggcgccggcatctgtgccagctaccagactcagacaaatagccctaggagagcaagatccgtggccagccagagcatcatcgcctatacaatgagcctgggcgccgagaattctgtcgcctacagcaacaacagcatcgccatccccactaatttcaccatctccgtcaccacagaaatcctgcctgtgagcatgaccaagaccagcgtggattgcacaatgtacatttgcggcgacagcaccgagtgttccaacctgctgctgcagtacggcagcttctgcacccagctgaacagagcactgacaggcatcgccgtggagcaagacaagaacacccaggaggtgttcgcccaggtgaagcagatctacaagacccctcctatcaaagacttcggtggcttcaacttcagccagatcctgcctgatccgagcaagcctagcaaaagatcatttatcgaagacctgctgtttaacaaggtgaccctggccgacgccggattcatcaagcagtacggcgactgcctgggcgacatcgccgccagagatctgatctgtgcccagaagtttaatggcctgaccgtgctgccacctctgctgaccgacgagatgatcgcccaatataccagcgccctgctggctggaacaatcacaagcggctggaccttcggagccggagccgctcttcagattcctttcgccatgcagatggcctacagattcaacggcatcggcgtgacccagaacgtgctgtatgagaaccagaaactgatcgctaatcaatttaacagcgccatcggcaagattcaggactccctgagctcaacagcctctgccctgggcaagctgcaggatgtggtgaaccagaacgcccaggccctgaacacactggtgaaacagctgtcaagcaacttcggcgccatctcatccgtactgaacgacatcctgtctagactcgatccaccagaggccgaagtgcagatcgacagactgatcaccggccggctgcagagcctgcagacgtacgtgacccaacagctgatcagggccgccgagatccgggcctcggctaatttggccgccaccaaaatgagcgaatgcgtgctgggccagtctaagagggtcgacttctgtggcaagggctaccacctgatgagcttcccccagagcgctccccacggcgtggtgttcctgcacgtgacctacgttccagcccaggagaagaactttacaaccgcccctgccatctgccacgacggcaaggcccacttccctagagagggagtctttgtgagcaatggcacccactggttcgttacccagagaaacttctacgagccccagatcatcaccacagacaacaccttcgtgagcggaaactgtgacgtggtgatcggcatcgtgaacaacaccgtgtacgaccccctgcaacccgagctggacagcttcaaggaagagctggacaaatactttaagaaccacacctcacctgacgtggacctgggagatatcagcggcataaatgcctccgtggtgaacatccagaaggaaatcgatagactcaatgaggtggctaagaacctgaacgaaagcctgatcgacctccaagagctgggcaaatacgagcagtacatcaagtggccttggtacatttggctgggctttatcgccggcctcatcgctatcgtgatggtgaccatcatgctgtgctgcatgacctcctgctgcagctgcctgaagggctgttgcagctgcggcagctgctgcaagttcgacgaagatgattctgaaccagtgctgaaaggcgtgaaactgcactacacctga

SEQ ID NO: 33 - RNA, 3888 nt, Artificial Sequence
  IFN-r SP - SARS-CoV-2 S
atgaagtacacttcttacattttggctttccaattgtgtatcgttttgggttccttaggttgttactgtttcgtgttcctcgtcttgctacctttggtttcttctcaatgtgttaatttgactaccagaacccaattaccaccagcttacaccaattcttttaccagaggcgtgtactaccccgacaaggtgttccggagtagcgtgctgcacagcacgcaggacctgttcctgccatttttctctaatgtgacctggtttcacgccatccacgtgtccggcacaaacggcacaaagcggttcgacaaccccgtgctgccattcaacgatggcgtgtacttcgcctctacagaaaagtccaatatcattaggggctggatcttcggaacaacgctggactcaaagacccagagcctgctgatcgtcaataacgccacaaatgtggtcattaaagtgtgcgaattccagttctgcaacgaccccttcctgggcgtctactatcataagaacaacaagtcttggatggaaagcgagttccgggtgtacagcagcgctaacaactgcaccttcgagtacgtttcccaacctttcctgatggacctggaaggcaagcagggcaatttcaagaacctgagagaattcgtgttcaagaacatcgacggctacttcaagatctacagcaagcacacccccatcaacctggtacgagatctgccccagggcttctctgccctcgagcccctcgtggacctgcccattggaatcaacatcacgcggttccagaccctgctcgccctgcatagaagctacctcactcccggcgattctagcagcggctggacagccggcgctgccgcttactacgtgggctacctgcagcctagaacatttctactgaagtataacgagaacgggacaatcacagacgccgtggactgcgctctggatcctctgagcgaaaccaagtgcaccctgaaaagcttcaccgtcgagaagggaatctaccagacctccaacttccgggtgcagccaaccgagagcatcgtgagattccctaacatcactaacctgtgtccttttggagaagtgttcaacgccacccggttcgccagcgtttatgcctggaaccgcaagagaatctctaactgtgtggccgactacagcgtgctgtacaattctgccagcttcagcaccttcaagtgctacggcgtgagtcccaccaaactgaacgacctgtgcttcactaacgtgtacgccgatagctttgtgatcagaggagacgaggtgagacagattgctcctggccagaccggcaaaatcgccgattacaactacaagctacctgacgacttcaccggctgcgtgatcgcctggaattctaacaacctggactccaaggtgggcggcaactacaactacctgtacagactgtttcggaagtccaacctgaaaccattcgagagagatatcagcacagagatctaccaagcgggctcgacaccttgcaacggagtggagggcttcaactgttactttcctctgcagtcttatggcttccaacctacaaatggcgtcggatatcagccctacagagtggtggtgctttctttcgagctgctgcacgccccagctaccgtgtgtggtcctaagaagtcgacaaatctggtgaagaataagtgcgtgaattttaactttaacggcctgaccggcaccggcgtgctgaccgaatctaacaagaaattcctgcctttccagcagttcggtagagatatcgccgacaccaccgatgccgtgcgggaccctcaaacactggaaatcctggacataacaccttgcagcttcggcggagtcagcgtgatcacacctggcaccaacaccagcaaccaggtggccgtgctgtaccaggacgtgaactgcacagaagtgcctgtggcgatccacgctgatcagctgacacctacatggcgggtgtactcaacaggaagcaacgtgtttcagacacgggccggctgtctgatcggcgctgaacacgttaacaacagctacgagtgcgacatccccatcggcgccggcatctgtgccagctaccagactcagacaaatagccctaggagagcaagatccgtggccagccagagcatcatcgcctatacaatgagcctgggcgccgagaattctgtcgcctacagcaacaacagcatcgccatccccactaatttcaccatctccgtcaccacagaaatcctgcctgtgagcatgaccaagaccagcgtggattgcacaatgtacatttgcggcgacagcaccgagtgttccaacctgctgctgcagtacggcagcttctgcacccagctgaacagagcactgacaggcatcgccgtggagcaagacaagaacacccaggaggtgttcgcccaggtgaagcagatctacaagacccctcctatcaaagacttcggtggcttcaacttcagccagatcctgcctgatccgagcaagcctagcaaaagatcatttatcgaagacctgctgtttaacaaggtgaccctggccgacgccggattcatcaagcagtacggcgactgcctgggcgacatcgccgccagagatctgatctgtgcccagaagtttaatggcctgaccgtgctgccacctctgctgaccgacgagatgatcgcccaatataccagcgccctgctggctggaacaatcacaagcggctggaccttcggagccggagccgctcttcagattcctttcgccatgcagatggcctacagattcaacggcatcggcgtgacccagaacgtgctgtatgagaaccagaaactgatcgctaatcaatttaacagcgccatcggcaagattcaggactccctgagctcaacagcctctgccctgggcaagctgcaggatgtggtgaaccagaacgcccaggccctgaacacactggtgaaacagctgtcaagcaacttcggcgccatctcatccgtactgaacgacatcctgtctagactcgatccaccagaggccgaagtgcagatcgacagactgatcaccggccggctgcagagcctgcagacgtacgtgacccaacagctgatcagggccgccgagatccgggcctcggctaatttggccgccaccaaaatgagcgaatgcgtgctgggccagtctaagagggtcgacttctgtggcaagggctaccacctgatgagcttcccccagagcgctccccacggcgtggtgttcctgcacgtgacctacgttccagcccaggagaagaactttacaaccgcccctgccatctgccacgacggcaaggcccacttccctagagagggagtctttgtgagcaatggcacccactggttcgttacccagagaaacttctacgagccccagatcatcaccacagacaacaccttcgtgagcggaaactgtgacgtggtgatcggcatcgtgaacaacaccgtgtacgaccccctgcaacccgagctggacagcttcaaggaagagctggacaaatactttaagaaccacacctcacctgacgtggacctgggagatatcagcggcataaatgcctccgtggtgaacatccagaaggaaatcgatagactcaatgaggtggctaagaacctgaacgaaagcctgatcgacctccaagagctgggcaaatacgagcagtacatcaagtggccttggtacatttggctgggctttatcgccggcctcatcgctatcgtgatggtgaccatcatgctgtgctgcatgacctcctgctgcagctgcctgaagggctgttgcagctgcggcagctgctgcaagttcgacgaagatgattctgaaccagtgctgaaaggcgtgaaactgcactacacctga

SEQ ID NO: 34 - RNA, 3903 nt, Artificial Sequence
  F IX SP - SARS-CoV-2 S
atgcaaagagttaacatgattatggctgaatctccaggtttgatcactatctgtttgttgggttacttgttatccgccgaatgtttcgtgttcctcgtcttgctacctttggtttcttctcaatgtgttaatttgactaccagaacccaattaccaccagcttacaccaattcttttaccagaggcgtgtactaccccgacaaggtgttccggagtagcgtgctgcacagcacgcaggacctgttcctgccatttttctctaatgtgacctggtttcacgccatccacgtgtccggcacaaacggcacaaagcggttcgacaaccccgtgctgccattcaacgatggcgtgtacttcgcctctacagaaaagtccaatatcattaggggctggatcttcggaacaacgctggactcaaagacccagagcctgctgatcgtcaataacgccacaaatgtggtcattaaagtgtgcgaattccagttctgcaacgaccccttcctgggcgtctactatcataagaacaacaagtcttggatggaaagcgagttccgggtgtacagcagcgctaacaactgcaccttcgagtacgtttcccaacctttcctgatggacctggaaggcaagcagggcaatttcaagaacctgagagaattcgtgttcaagaacatcgacggctacttcaagatctacagcaagcacacccccatcaacctggtacgagatctgccccagggcttctctgccctcgagcccctcgtggacctgcccattggaatcaacatcacgcggttccagaccctgctcgccctgcatagaagctacctcactcccggcgattctagcagcggctggacagccggcgctgccgcttactacgtgggctacctgcagcctagaacatttctactgaagtataacgagaacgggacaatcacagacgccgtggactgcgctctggatcctctgagcgaaaccaagtgcaccctgaaaagcttcaccgtcgagaagggaatctaccagacctccaacttccgggtgcagccaaccgagagcatcgtgagattccctaacatcactaacctgtgtccttttggagaagtgttcaacgccacccggttcgccagcgtttatgcctggaaccgcaagagaatctctaactgtgtggccgactacagcgtgctgtacaattctgccagcttcagcaccttcaagtgctacggcgtgagtcccaccaaactgaacgacctgtgcttcactaacgtgtacgccgatagctttgtgatcagaggagacgaggtgagacagattgctcctggccagaccggcaaaatcgccgattacaactacaagctacctgacgacttcaccggctgcgtgatcgcctggaattctaacaacctggactccaaggtgggcggcaactacaactacctgtacagactgtttcggaagtccaacctgaaaccattcgagagagatatcagcacagagatctaccaagcgggctcgacaccttgcaacggagtggagggcttcaactgttactttcctctgcagtcttatggcttccaacctacaaatggcgtcggatatcagccctacagagtggtggtgctttctttcgagctgctgcacgccccagctaccgtgtgtggtcctaagaagtcgacaaatctggtgaagaataagtgcgtgaattttaactttaacggcctgaccggcaccggcgtgctgaccgaatctaacaagaaattcctgcctttccagcagttcggtagagatatcgccgacaccaccgatgccgtgcgggaccctcaaacactggaaatcctggacataacaccttgcagcttcggcggagtcagcgtgatcacacctggcaccaacaccagcaaccaggtggccgtgctgtaccaggacgtgaactgcacagaagtgcctgtggcgatccacgctgatcagctgacacctacatggcgggtgtactcaacaggaagcaacgtgtttcagacacgggccggctgtctgatcggcgctgaacacgttaacaacagctacgagtgcgacatccccatcggcgccggcatctgtgccagctaccagactcagacaaatagccctaggagagcaagatccgtggccagccagagcatcatcgcctatacaatgagcctgggcgccgagaattctgtcgcctacagcaacaacagcatcgccatccccactaatttcaccatctccgtcaccacagaaatcctgcctgtgagcatgaccaagaccagcgtggattgcacaatgtacatttgcggcgacagcaccgagtgttccaacctgctgctgcagtacggcagcttctgcacccagctgaacagagcactgacaggcatcgccgtggagcaagacaagaacacccaggaggtgttcgcccaggtgaagcagatctacaagacccctcctatcaaagacttcggtggcttcaacttcagccagatcctgcctgatccgagcaagcctagcaaaagatcatttatcgaagacctgctgtttaacaaggtgaccctggccgacgccggattcatcaagcagtacggcgactgcctgggcgacatcgccgccagagatctgatctgtgcccagaagtttaatggcctgaccgtgctgccacctctgctgaccgacgagatgatcgcccaatataccagcgccctgctggctggaacaatcacaagcggctggaccttcggagccggagccgctcttcagattcctttcgccatgcagatggcctacagattcaacggcatcggcgtgacccagaacgtgctgtatgagaaccagaaactgatcgctaatcaatttaacagcgccatcggcaagattcaggactccctgagctcaacagcctctgccctgggcaagctgcaggatgtggtgaaccagaacgcccaggccctgaacacactggtgaaacagctgtcaagcaacttcggcgccatctcatccgtactgaacgacatcctgtctagactcgatccaccagaggccgaagtgcagatcgacagactgatcaccggccggctgcagagcctgcagacgtacgtgacccaacagctgatcagggccgccgagatccgggcctcggctaatttggccgccaccaaaatgagcgaatgcgtgctgggccagtctaagagggtcgacttctgtggcaagggctaccacctgatgagcttcccccagagcgctccccacggcgtggtgttcctgcacgtgacctacgttccagcccaggagaagaactttacaaccgcccctgccatctgccacgacggcaaggcccacttccctagagagggagtctttgtgagcaatggcacccactggttcgttacccagagaaacttctacgagccccagatcatcaccacagacaacaccttcgtgagcggaaactgtgacgtggtgatcggcatcgtgaacaacaccgtgtacgaccccctgcaacccgagctggacagcttcaaggaagagctggacaaatactttaagaaccacacctcacctgacgtggacctgggagatatcagcggcataaatgcctccgtggtgaacatccagaaggaaatcgatagactcaatgaggtggctaagaacctgaacgaaagcctgatcgacctccaagagctgggcaaatacgagcagtacatcaagtggccttggtacatttggctgggctttatcgccggcctcatcgctatcgtgatggtgaccatcatgctgtgctgcatgacctcctgctgcagctgcctgaagggctgttgcagctgcggcagctgctgcaagttcgacgaagatgattctgaaccagtgctgaaaggcgtgaaactgcactacacctga

SEQ ID NO: 35 - RNA, 3879 nt, Artificial Sequence
  MLP1 SP - SARS-CoV-2 S
atggtatataaaactttatttgctttatgtattttaactgctggttggcgtgtacaatctttcgtgttcctcgtcttgctacctttggtttcttctcaatgtgttaatttgactaccagaacccaattaccaccagcttacaccaattcttttaccagaggcgtgtactaccccgacaaggtgttccggagtagcgtgctgcacagcacgcaggacctgttcctgccatttttctctaatgtgacctggtttcacgccatccacgtgtccggcacaaacggcacaaagcggttcgacaaccccgtgctgccattcaacgatggcgtgtacttcgcctctacagaaaagtccaatatcattaggggctggatcttcggaacaacgctggactcaaagacccagagcctgctgatcgtcaataacgccacaaatgtggtcattaaagtgtgcgaattccagttctgcaacgaccccttcctgggcgtctactatcataagaacaacaagtcttggatggaaagcgagttccgggtgtacagcagcgctaacaactgcaccttcgagtacgtttcccaacctttcctgatggacctggaaggcaagcagggcaatttcaagaacctgagagaattcgtgttcaagaacatcgacggctacttcaagatctacagcaagcacacccccatcaacctggtacgagatctgccccagggcttctctgccctcgagcccctcgtggacctgcccattggaatcaacatcacgcggttccagaccctgctcgccctgcatagaagctacctcactcccggcgattctagcagcggctggacagccggcgctgccgcttactacgtgggctacctgcagcctagaacatttctactgaagtataacgagaacgggacaatcacagacgccgtggactgcgctctggatcctctgagcgaaaccaagtgcaccctgaaaagcttcaccgtcgagaagggaatctaccagacctccaacttccgggtgcagccaaccgagagcatcgtgagattccctaacatcactaacctgtgtccttttggagaagtgttcaacgccacccggttcgccagcgtttatgcctggaaccgcaagagaatctctaactgtgtggccgactacagcgtgctgtacaattctgccagcttcagcaccttcaagtgctacggcgtgagtcccaccaaactgaacgacctgtgcttcactaacgtgtacgccgatagctttgtgatcagaggagacgaggtgagacagattgctcctggccagaccggcaaaatcgccgattacaactacaagctacctgacgacttcaccggctgcgtgatcgcctggaattctaacaacctggactccaaggtgggcggcaactacaactacctgtacagactgtttcggaagtccaacctgaaaccattcgagagagatatcagcacagagatctaccaagcgggctcgacaccttgcaacggagtggagggcttcaactgttactttcctctgcagtcttatggcttccaacctacaaatggcgtcggatatcagccctacagagtggtggtgctttctttcgagctgctgcacgccccagctaccgtgtgtggtcctaagaagtcgacaaatctggtgaagaataagtgcgtgaattttaactttaacggcctgaccggcaccggcgtgctgaccgaatctaacaagaaattcctgcctttccagcagttcggtagagatatcgccgacaccaccgatgccgtgcgggaccctcaaacactggaaatcctggacataacaccttgcagcttcggcggagtcagcgtgatcacacctggcaccaacaccagcaaccaggtggccgtgctgtaccaggacgtgaactgcacagaagtgcctgtggcgatccacgctgatcagctgacacctacatggcgggtgtactcaacaggaagcaacgtgtttcagacacgggccggctgtctgatcggcgctgaacacgttaacaacagctacgagtgcgacatccccatcggcgccggcatctgtgccagctaccagactcagacaaatagccctaggagagcaagatccgtggccagccagagcatcatcgcctatacaatgagcctgggcgccgagaattctgtcgcctacagcaacaacagcatcgccatccccactaatttcaccatctccgtcaccacagaaatcctgcctgtgagcatgaccaagaccagcgtggattgcacaatgtacatttgcggcgacagcaccgagtgttccaacctgctgctgcagtacggcagcttctgcacccagctgaacagagcactgacaggcatcgccgtggagcaagacaagaacacccaggaggtgttcgcccaggtgaagcagatctacaagacccctcctatcaaagacttcggtggcttcaacttcagccagatcctgcctgatccgagcaagcctagcaaaagatcatttatcgaagacctgctgtttaacaaggtgaccctggccgacgccggattcatcaagcagtacggcgactgcctgggcgacatcgccgccagagatctgatctgtgcccagaagtttaatggcctgaccgtgctgccacctctgctgaccgacgagatgatcgcccaatataccagcgccctgctggctggaacaatcacaagcggctggaccttcggagccggagccgctcttcagattcctttcgccatgcagatggcctacagattcaacggcatcggcgtgacccagaacgtgctgtatgagaaccagaaactgatcgctaatcaatttaacagcgccatcggcaagattcaggactccctgagctcaacagcctctgccctgggcaagctgcaggatgtggtgaaccagaacgcccaggccctgaacacactggtgaaacagctgtcaagcaacttcggcgccatctcatccgtactgaacgacatcctgtctagactcgatccaccagaggccgaagtgcagatcgacagactgatcaccggccggctgcagagcctgcagacgtacgtgacccaacagctgatcagggccgccgagatccgggcctcggctaatttggccgccaccaaaatgagcgaatgcgtgctgggccagtctaagagggtcgacttctgtggcaagggctaccacctgatgagcttcccccagagcgctccccacggcgtggtgttcctgcacgtgacctacgttccagcccaggagaagaactttacaaccgcccctgccatctgccacgacggcaaggcccacttccctagagagggagtctttgtgagcaatggcacccactggttcgttacccagagaaacttctacgagccccagatcatcaccacagacaacaccttcgtgagcggaaactgtgacgtggtgatcggcatcgtgaacaacaccgtgtacgaccccctgcaacccgagctggacagcttcaaggaagagctggacaaatactttaagaaccacacctcacctgacgtggacctgggagatatcagcggcataaatgcctccgtggtgaacatccagaaggaaatcgatagactcaatgaggtggctaagaacctgaacgaaagcctgatcgacctccaagagctgggcaaatacgagcagtacatcaagtggccttggtacatttggctgggctttatcgccggcctcatcgctatcgtgatggtgaccatcatgctgtgctgcatgacctcctgctgcagctgcctgaagggctgttgcagctgcggcagctgctgcaagttcgacgaagatgattctgaaccagtgctgaaaggcgtgaaactgcactacacctga

SEQ ID NO: 36 - RNA, 720 nt, Artificial Sequence
  albumin SP - SARS-CoV-2 M
atgaagtgggtaacctttatttcccttctttttctctttagctcggcttattccgctgattccaacggtaccatcaccgttgaagaattgaagaagttgctggaacaatggaacttggtcattggttttttattcttgacttggatctgtttgttgcaattcgcttacgctaacagaaaccgtttcctctacattatcaagttgatcttcctatggttattgtggccagtcactttggcttgtttcgttttggccgcagtttacagaatcaactggattacaggtggtattgctattgctatggcctgtctggtgggcctgatgtggctgagctacttcatcgcctcttttagactgtttgccagaacccggagcatgtggtccttcaaccccgagacaaacatcctgctgaatgtgcccctgcacggcacaatcctgacaagacctctgcttgagagcgagctggtgatcggcgccgtgatcctgaggggccatctgcggattgccggacaccacctgggcagatgcgacatcaaggacctgcctaaggaaatcaccgtggctacaagccgcaccctgtcctactacaaactcggcgccagccaaagagtggccggcgacagcggcttcgccgcctatagcagataccggatcggcaactacaagctgaacaccgaccactctagcagctctgataatatcgccctgctggttcagtga

SEQ ID NO: 37 - RNA, 720 nt, Artificial Sequence
  albumin SP - SARS-CoV-2 M
atgaagtgggttactttcatctctttgttgtttttattctcctctgcttactccgctgattccaacggtaccatcaccgttgaagaattgaagaagttgctggaacaatggaacttggtcattggttttttattcttgacttggatctgtttgttgcaattcgcttacgctaacagaaaccgtttcctctacattatcaagttgatcttcctatggttattgtggccagtcactttggcttgtttcgttttggccgcagtttacagaatcaactggattacaggtggtattgctattgctatggcctgtctggtgggcctgatgtggctgagctacttcatcgcctcttttagactgtttgccagaacccggagcatgtggtccttcaaccccgagacaaacatcctgctgaatgtgcccctgcacggcacaatcctgacaagacctctgcttgagagcgagctggtgatcggcgccgtgatcctgaggggccatctgcggattgccggacaccacctgggcagatgcgacatcaaggacctgcctaaggaaatcaccgtggctacaagccgcaccctgtcctactacaaactcggcgccagccaaagagtggccggcgacagcggcttcgccgcctatagcagataccggatcggcaactacaagctgaacaccgaccactctagcagctctgataatatcgccctgctggttcagtga

SEQ ID NO: 38 - RNA, 735 nt, Artificial Sequence
  IFN-r SP - SARS-CoV-2 M
atgaaatatacaagttatatcttggcttttcagctctgcatcgttttgggttctcttggctgttactgcgctgattccaacggtaccatcaccgttgaagaattgaagaagttgctggaacaatggaacttggtcattggttttttattcttgacttggatctgtttgttgcaattcgcttacgctaacagaaaccgtttcctctacattatcaagttgatcttcctatggttattgtggccagtcactttggcttgtttcgttttggccgcagtttacagaatcaactggattacaggtggtattgctattgctatggcctgtctggtgggcctgatgtggctgagctacttcatcgcctcttttagactgtttgccagaacccggagcatgtggtccttcaaccccgagacaaacatcctgctgaatgtgcccctgcacggcacaatcctgacaagacctctgcttgagagcgagctggtgatcggcgccgtgatcctgaggggccatctgcggattgccggacaccacctgggcagatgcgacatcaaggacctgcctaaggaaatcaccgtggctacaagccgcaccctgtcctactacaaactcggcgccagccaaagagtggccggcgacagcggcttcgccgcctatagcagataccggatcggcaactacaagctgaacaccgaccactctagcagctctgataatatcgccctgctggttcagtga

SEQ ID NO: 39 - RNA, 735 nt, Artificial Sequence
  IFN-r SP - SARS-CoV-2 M
atgaagtacacttcttacattttggctttccaattgtgtatcgttttgggttccttaggttgttactgtgctgattccaacggtaccatcaccgttgaagaattgaagaagttgctggaacaatggaacttggtcattggttttttattcttgacttggatctgtttgttgcaattcgcttacgctaacagaaaccgtttcctctacattatcaagttgatcttcctatggttattgtggccagtcactttggcttgtttcgttttggccgcagtttacagaatcaactggattacaggtggtattgctattgctatggcctgtctggtgggcctgatgtggctgagctacttcatcgcctcttttagactgtttgccagaacccggagcatgtggtccttcaaccccgagacaaacatcctgctgaatgtgcccctgcacggcacaatcctgacaagacctctgcttgagagcgagctggtgatcggcgccgtgatcctgaggggccatctgcggattgccggacaccacctgggcagatgcgacatcaaggacctgcctaaggaaatcaccgtggctacaagccgcaccctgtcctactacaaactcggcgccagccaaagagtggccggcgacagcggcttcgccgcctatagcagataccggatcggcaactacaagctgaacaccgaccactctagcagctctgataatatcgccctgctggttcagtga

SEQ ID NO: 40 - RNA, 750 nt, Artificial Sequence
  F IX SP - SARS-CoV-2 M
atgcagcgcgtgaacatgatcatggcagaatcaccaggcctcatcaccatctgccttttaggatatctactcagtgctgaatgtgctgattccaacggtaccatcaccgttgaagaattgaagaagttgctggaacaatggaacttggtcattggttttttattcttgacttggatctgtttgttgcaattcgcttacgctaacagaaaccgtttcctctacattatcaagttgatcttcctatggttattgtggccagtcactttggcttgtttcgttttggccgcagtttacagaatcaactggattacaggtggtattgctattgctatggcctgtctggtgggcctgatgtggctgagctacttcatcgcctcttttagactgtttgccagaacccggagcatgtggtccttcaaccccgagacaaacatcctgctgaatgtgcccctgcacggcacaatcctgacaagacctctgcttgagagcgagctggtgatcggcgccgtgatcctgaggggccatctgcggattgccggacaccacctgggcagatgcgacatcaaggacctgcctaaggaaatcaccgtggctacaagccgcaccctgtcctactacaaactcggcgccagccaaagagtggccggcgacagcggcttcgccgcctatagcagataccggatcggcaactacaagctgaacaccgaccactctagcagctctgataatatcgccctgctggttcagtga

SEQ ID NO: 41 - RNA, 750 nt, Artificial Sequence
  F IX SP - SARS-CoV-2 M
atgcaaagagttaacatgattatggctgaatctccaggtttgatcactatctgtttgttgggttacttgttatccgccgaatgtgctgattccaacggtaccatcaccgttgaagaattgaagaagttgctggaacaatggaacttggtcattggttttttattcttgacttggatctgtttgttgcaattcgcttacgctaacagaaaccgtttcctctacattatcaagttgatcttcctatggttattgtggccagtcactttggcttgtttcgttttggccgcagtttacagaatcaactggattacaggtggtattgctattgctatggcctgtctggtgggcctgatgtggctgagctacttcatcgcctcttttagactgtttgccagaacccggagcatgtggtccttcaaccccgagacaaacatcctgctgaatgtgcccctgcacggcacaatcctgacaagacctctgcttgagagcgagctggtgatcggcgccgtgatcctgaggggccatctgcggattgccggacaccacctgggcagatgcgacatcaaggacctgcctaaggaaatcaccgtggctacaagccgcaccctgtcctactacaaactcggcgccagccaaagagtggccggcgacagcggcttcgccgcctatagcagataccggatcggcaactacaagctgaacaccgaccactctagcagctctgataatatcgccctgctggttcagtga

SEQ ID NO: 42 - RNA, 726 nt, Artificial Sequence
  MLP1 SP - SARS-CoV-2 M
atggtctacaagactctcttcgctctttgcatcttaactgcaggatggagggtacagagtgctgattccaacggtaccatcaccgttgaagaattgaagaagttgctggaacaatggaacttggtcattggttttttattcttgacttggatctgtttgttgcaattcgcttacgctaacagaaaccgtttcctctacattatcaagttgatcttcctatggttattgtggccagtcactttggcttgtttcgttttggccgcagtttacagaatcaactggattacaggtggtattgctattgctatggcctgtctggtgggcctgatgtggctgagctacttcatcgcctcttttagactgtttgccagaacccggagcatgtggtccttcaaccccgagacaaacatcctgctgaatgtgcccctgcacggcacaatcctgacaagacctctgcttgagagcgagctggtgatcggcgccgtgatcctgaggggccatctgcggattgccggacaccacctgggcagatgcgacatcaaggacctgcctaaggaaatcaccgtggctacaagccgcaccctgtcctactacaaactcggcgccagccaaagagtggccggcgacagcggcttcgccgcctatagcagataccggatcggcaactacaagctgaacaccgaccactctagcagctctgataatatcgccctgctggttcagtga

SEQ ID NO: 43 - RNA, 726 nt, Artificial Sequence
  MLP1 SP - SARS-CoV-2 M
atggtatataaaactttatttgctttatgtattttaactgctggttggcgtgtacaatctgctgattccaacggtaccatcaccgttgaagaattgaagaagttgctggaacaatggaacttggtcattggttttttattcttgacttggatctgtttgttgcaattcgcttacgctaacagaaaccgtttcctctacattatcaagttgatcttcctatggttattgtggccagtcactttggcttgtttcgttttggccgcagtttacagaatcaactggattacaggtggtattgctattgctatggcctgtctggtgggcctgatgtggctgagctacttcatcgcctcttttagactgtttgccagaacccggagcatgtggtccttcaaccccgagacaaacatcctgctgaatgtgcccctgcacggcacaatcctgacaagacctctgcttgagagcgagctggtgatcggcgccgtgatcctgaggggccatctgcggattgccggacaccacctgggcagatgcgacatcaaggacctgcctaaggaaatcaccgtggctacaagccgcaccctgtcctactacaaactcggcgccagccaaagagtggccggcgacagcggcttcgccgcctatagcagataccggatcggcaactacaagctgaacaccgaccactctagcagctctgataatatcgccctgctggttcagtga

SEQ ID NO: 44 - protein, 48 aa, Artificial Sequence
  TTTh
RQKRIDKISDVSTIVPYIGPALNIPKKRNNFTVSFWLRVPKVSASHLE

SEQ ID NO: 45 - RNA, 147 nt, Artificial Sequence
  TTTh
cgccagaaacgcattgataaaattagcgatgtgagcaccattgtgccgtatattggcccggcgctgaacattccgaaaaaacgcaacaactttaccgtgagcttttggctgcgcgtgccgaaagtgagcgcgagccatctggaatga

SEQ ID NO: 46 - RNA, 147 nt, Artificial Sequence
  TTTh
agacagaaaagaatcgataagatcagcgacgtgtctacaatcgtgccatacatcggccctgccctgaatatccccaagaagcggaacaacttcaccgtcagcttctggctgagagtgcctaaggtgtccgccagccacctggagtga

SEQ ID NO: 47 - RNA, 4017 nt, Artificial Sequence
  IgE SP - SARS-CoV-2 S - TTTh
atggactggacttggatcttgttcttggttgctgctgccaccagagtccactctttcgtgttcctcgtcttgctacctttggtttcttctcaatgtgttaatttgactaccagaacccaattaccaccagcttacaccaattcttttaccagaggcgtgtactaccccgacaaggtgttccggagtagcgtgctgcacagcacgcaggacctgttcctgccatttttctctaatgtgacctggtttcacgccatccacgtgtccggcacaaacggcacaaagcggttcgacaaccccgtgctgccattcaacgatggcgtgtacttcgcctctacagaaaagtccaatatcattaggggctggatcttcggaacaacgctggactcaaagacccagagcctgctgatcgtcaataacgccacaaatgtggtcattaaagtgtgcgaattccagttctgcaacgaccccttcctgggcgtctactatcataagaacaacaagtcttggatggaaagcgagttccgggtgtacagcagcgctaacaactgcaccttcgagtacgtttcccaacctttcctgatggacctggaaggcaagcagggcaatttcaagaacctgagagaattcgtgttcaagaacatcgacggctacttcaagatctacagcaagcacacccccatcaacctggtacgagatctgccccagggcttctctgccctcgagcccctcgtggacctgcccattggaatcaacatcacgcggttccagaccctgctcgccctgcatagaagctacctcactcccggcgattctagcagcggctggacagccggcgctgccgcttactacgtgggctacctgcagcctagaacatttctactgaagtataacgagaacgggacaatcacagacgccgtggactgcgctctggatcctctgagcgaaaccaagtgcaccctgaaaagcttcaccgtcgagaagggaatctaccagacctccaacttccgggtgcagccaaccgagagcatcgtgagattccctaacatcactaacctgtgtccttttggagaagtgttcaacgccacccggttcgccagcgtttatgcctggaaccgcaagagaatctctaactgtgtggccgactacagcgtgctgtacaattctgccagcttcagcaccttcaagtgctacggcgtgagtcccaccaaactgaacgacctgtgcttcactaacgtgtacgccgatagctttgtgatcagaggagacgaggtgagacagattgctcctggccagaccggcaaaatcgccgattacaactacaagctacctgacgacttcaccggctgcgtgatcgcctggaattctaacaacctggactccaaggtgggcggcaactacaactacctgtacagactgtttcggaagtccaacctgaaaccattcgagagagatatcagcacagagatctaccaagcgggctcgacaccttgcaacggagtggagggcttcaactgttactttcctctgcagtcttatggcttccaacctacaaatggcgtcggatatcagccctacagagtggtggtgctttctttcgagctgctgcacgccccagctaccgtgtgtggtcctaagaagtcgacaaatctggtgaagaataagtgcgtgaattttaactttaacggcctgaccggcaccggcgtgctgaccgaatctaacaagaaattcctgcctttccagcagttcggtagagatatcgccgacaccaccgatgccgtgcgggaccctcaaacactggaaatcctggacataacaccttgcagcttcggcggagtcagcgtgatcacacctggcaccaacaccagcaaccaggtggccgtgctgtaccaggacgtgaactgcacagaagtgcctgtggcgatccacgctgatcagctgacacctacatggcgggtgtactcaacaggaagcaacgtgtttcagacacgggccggctgtctgatcggcgctgaacacgttaacaacagctacgagtgcgacatccccatcggcgccggcatctgtgccagctaccagactcagacaaatagccctaggagagcaagatccgtggccagccagagcatcatcgcctatacaatgagcctgggcgccgagaattctgtcgcctacagcaacaacagcatcgccatccccactaatttcaccatctccgtcaccacagaaatcctgcctgtgagcatgaccaagaccagcgtggattgcacaatgtacatttgcggcgacagcaccgagtgttccaacctgctgctgcagtacggcagcttctgcacccagctgaacagagcactgacaggcatcgccgtggagcaagacaagaacacccaggaggtgttcgcccaggtgaagcagatctacaagacccctcctatcaaagacttcggtggcttcaacttcagccagatcctgcctgatccgagcaagcctagcaaaagatcatttatcgaagacctgctgtttaacaaggtgaccctggccgacgccggattcatcaagcagtacggcgactgcctgggcgacatcgccgccagagatctgatctgtgcccagaagtttaatggcctgaccgtgctgccacctctgctgaccgacgagatgatcgcccaatataccagcgccctgctggctggaacaatcacaagcggctggaccttcggagccggagccgctcttcagattcctttcgccatgcagatggcctacagattcaacggcatcggcgtgacccagaacgtgctgtatgagaaccagaaactgatcgctaatcaatttaacagcgccatcggcaagattcaggactccctgagctcaacagcctctgccctgggcaagctgcaggatgtggtgaaccagaacgcccaggccctgaacacactggtgaaacagctgtcaagcaacttcggcgccatctcatccgtactgaacgacatcctgtctagactcgatccaccagaggccgaagtgcagatcgacagactgatcaccggccggctgcagagcctgcagacgtacgtgacccaacagctgatcagggccgccgagatccgggcctcggctaatttggccgccaccaaaatgagcgaatgcgtgctgggccagtctaagagggtcgacttctgtggcaagggctaccacctgatgagcttcccccagagcgctccccacggcgtggtgttcctgcacgtgacctacgttccagcccaggagaagaactttacaaccgcccctgccatctgccacgacggcaaggcccacttccctagagagggagtctttgtgagcaatggcacccactggttcgttacccagagaaacttctacgagccccagatcatcaccacagacaacaccttcgtgagcggaaactgtgacgtggtgatcggcatcgtgaacaacaccgtgtacgaccccctgcaacccgagctggacagcttcaaggaagagctggacaaatactttaagaaccacacctcacctgacgtggacctgggagatatcagcggcataaatgcctccgtggtgaacatccagaaggaaatcgatagactcaatgaggtggctaagaacctgaacgaaagcctgatcgacctccaagagctgggcaaatacgagcagtacatcaagtggccttggtacatttggctgggctttatcgccggcctcatcgctatcgtgatggtgaccatcatgctgtgctgcatgacctcctgctgcagctgcctgaagggctgttgcagctgcggcagctgctgcaagttcgacgaagatgattctgaaccagtgctgaaaggcgtgaaactgcactacaccagacagaaaagaatcgataagatcagcgacgtgtctacaatcgtgccatacatcggccctgccctgaatatccccaagaagcggaacaacttcaccgtcagcttctggctgagagtgcctaaggtgtccgccagccacctggagtga

SEQ ID NO: 48 - RNA, 4017 nt, Artificial Sequence
  albumin SP - SARS-CoV-2 S - TTTh
atgaagtgggttactttcatctctttgttgtttttattctcctctgcttactccttcgtgttcctcgtcttgctacctttggtttcttctcaatgtgttaatttgactaccagaacccaattaccaccagcttacaccaattcttttaccagaggcgtgtactaccccgacaaggtgttccggagtagcgtgctgcacagcacgcaggacctgttcctgccatttttctctaatgtgacctggtttcacgccatccacgtgtccggcacaaacggcacaaagcggttcgacaaccccgtgctgccattcaacgatggcgtgtacttcgcctctacagaaaagtccaatatcattaggggctggatcttcggaacaacgctggactcaaagacccagagcctgctgatcgtcaataacgccacaaatgtggtcattaaagtgtgcgaattccagttctgcaacgaccccttcctgggcgtctactatcataagaacaacaagtcttggatggaaagcgagttccgggtgtacagcagcgctaacaactgcaccttcgagtacgtttcccaacctttcctgatggacctggaaggcaagcagggcaatttcaagaacctgagagaattcgtgttcaagaacatcgacggctacttcaagatctacagcaagcacacccccatcaacctggtacgagatctgccccagggcttctctgccctcgagcccctcgtggacctgcccattggaatcaacatcacgcggttccagaccctgctcgccctgcatagaagctacctcactcccggcgattctagcagcggctggacagccggcgctgccgcttactacgtgggctacctgcagcctagaacatttctactgaagtataacgagaacgggacaatcacagacgccgtggactgcgctctggatcctctgagcgaaaccaagtgcaccctgaaaagcttcaccgtcgagaagggaatctaccagacctccaacttccgggtgcagccaaccgagagcatcgtgagattccctaacatcactaacctgtgtccttttggagaagtgttcaacgccacccggttcgccagcgtttatgcctggaaccgcaagagaatctctaactgtgtggccgactacagcgtgctgtacaattctgccagcttcagcaccttcaagtgctacggcgtgagtcccaccaaactgaacgacctgtgcttcactaacgtgtacgccgatagctttgtgatcagaggagacgaggtgagacagattgctcctggccagaccggcaaaatcgccgattacaactacaagctacctgacgacttcaccggctgcgtgatcgcctggaattctaacaacctggactccaaggtgggcggcaactacaactacctgtacagactgtttcggaagtccaacctgaaaccattcgagagagatatcagcacagagatctaccaagcgggctcgacaccttgcaacggagtggagggcttcaactgttactttcctctgcagtcttatggcttccaacctacaaatggcgtcggatatcagccctacagagtggtggtgctttctttcgagctgctgcacgccccagctaccgtgtgtggtcctaagaagtcgacaaatctggtgaagaataagtgcgtgaattttaactttaacggcctgaccggcaccggcgtgctgaccgaatctaacaagaaattcctgcctttccagcagttcggtagagatatcgccgacaccaccgatgccgtgcgggaccctcaaacactggaaatcctggacataacaccttgcagcttcggcggagtcagcgtgatcacacctggcaccaacaccagcaaccaggtggccgtgctgtaccaggacgtgaactgcacagaagtgcctgtggcgatccacgctgatcagctgacacctacatggcgggtgtactcaacaggaagcaacgtgtttcagacacgggccggctgtctgatcggcgctgaacacgttaacaacagctacgagtgcgacatccccatcggcgccggcatctgtgccagctaccagactcagacaaatagccctaggagagcaagatccgtggccagccagagcatcatcgcctatacaatgagcctgggcgccgagaattctgtcgcctacagcaacaacagcatcgccatccccactaatttcaccatctccgtcaccacagaaatcctgcctgtgagcatgaccaagaccagcgtggattgcacaatgtacatttgcggcgacagcaccgagtgttccaacctgctgctgcagtacggcagcttctgcacccagctgaacagagcactgacaggcatcgccgtggagcaagacaagaacacccaggaggtgttcgcccaggtgaagcagatctacaagacccctcctatcaaagacttcggtggcttcaacttcagccagatcctgcctgatccgagcaagcctagcaaaagatcatttatcgaagacctgctgtttaacaaggtgaccctggccgacgccggattcatcaagcagtacggcgactgcctgggcgacatcgccgccagagatctgatctgtgcccagaagtttaatggcctgaccgtgctgccacctctgctgaccgacgagatgatcgcccaatataccagcgccctgctggctggaacaatcacaagcggctggaccttcggagccggagccgctcttcagattcctttcgccatgcagatggcctacagattcaacggcatcggcgtgacccagaacgtgctgtatgagaaccagaaactgatcgctaatcaatttaacagcgccatcggcaagattcaggactccctgagctcaacagcctctgccctgggcaagctgcaggatgtggtgaaccagaacgcccaggccctgaacacactggtgaaacagctgtcaagcaacttcggcgccatctcatccgtactgaacgacatcctgtctagactcgatccaccagaggccgaagtgcagatcgacagactgatcaccggccggctgcagagcctgcagacgtacgtgacccaacagctgatcagggccgccgagatccgggcctcggctaatttggccgccaccaaaatgagcgaatgcgtgctgggccagtctaagagggtcgacttctgtggcaagggctaccacctgatgagcttcccccagagcgctccccacggcgtggtgttcctgcacgtgacctacgttccagcccaggagaagaactttacaaccgcccctgccatctgccacgacggcaaggcccacttccctagagagggagtctttgtgagcaatggcacccactggttcgttacccagagaaacttctacgagccccagatcatcaccacagacaacaccttcgtgagcggaaactgtgacgtggtgatcggcatcgtgaacaacaccgtgtacgaccccctgcaacccgagctggacagcttcaaggaagagctggacaaatactttaagaaccacacctcacctgacgtggacctgggagatatcagcggcataaatgcctccgtggtgaacatccagaaggaaatcgatagactcaatgaggtggctaagaacctgaacgaaagcctgatcgacctccaagagctgggcaaatacgagcagtacatcaagtggccttggtacatttggctgggctttatcgccggcctcatcgctatcgtgatggtgaccatcatgctgtgctgcatgacctcctgctgcagctgcctgaagggctgttgcagctgcggcagctgctgcaagttcgacgaagatgattctgaaccagtgctgaaaggcgtgaaactgcactacaccagacagaaaagaatcgataagatcagcgacgtgtctacaatcgtgccatacatcggccctgccctgaatatccccaagaagcggaacaacttcaccgtcagcttctggctgagagtgcctaaggtgtccgccagccacctggagtga

SEQ ID NO: 49 - RNA, 4032 nt, Artificial Sequence
  IFN-r SP - SARS-CoV-2 S - TTTh
atgaagtacacttcttacattttggctttccaattgtgtatcgttttgggttccttaggttgttactgtttcgtgttcctcgtcttgctacctttggtttcttctcaatgtgttaatttgactaccagaacccaattaccaccagcttacaccaattcttttaccagaggcgtgtactaccccgacaaggtgttccggagtagcgtgctgcacagcacgcaggacctgttcctgccatttttctctaatgtgacctggtttcacgccatccacgtgtccggcacaaacggcacaaagcggttcgacaaccccgtgctgccattcaacgatggcgtgtacttcgcctctacagaaaagtccaatatcattaggggctggatcttcggaacaacgctggactcaaagacccagagcctgctgatcgtcaataacgccacaaatgtggtcattaaagtgtgcgaattccagttctgcaacgaccccttcctgggcgtctactatcataagaacaacaagtcttggatggaaagcgagttccgggtgtacagcagcgctaacaactgcaccttcgagtacgtttcccaacctttcctgatggacctggaaggcaagcagggcaatttcaagaacctgagagaattcgtgttcaagaacatcgacggctacttcaagatctacagcaagcacacccccatcaacctggtacgagatctgccccagggcttctctgccctcgagcccctcgtggacctgcccattggaatcaacatcacgcggttccagaccctgctcgccctgcatagaagctacctcactcccggcgattctagcagcggctggacagccggcgctgccgcttactacgtgggctacctgcagcctagaacatttctactgaagtataacgagaacgggacaatcacagacgccgtggactgcgctctggatcctctgagcgaaaccaagtgcaccctgaaaagcttcaccgtcgagaagggaatctaccagacctccaacttccgggtgcagccaaccgagagcatcgtgagattccctaacatcactaacctgtgtccttttggagaagtgttcaacgccacccggttcgccagcgtttatgcctggaaccgcaagagaatctctaactgtgtggccgactacagcgtgctgtacaattctgccagcttcagcaccttcaagtgctacggcgtgagtcccaccaaactgaacgacctgtgcttcactaacgtgtacgccgatagctttgtgatcagaggagacgaggtgagacagattgctcctggccagaccggcaaaatcgccgattacaactacaagctacctgacgacttcaccggctgcgtgatcgcctggaattctaacaacctggactccaaggtgggcggcaactacaactacctgtacagactgtttcggaagtccaacctgaaaccattcgagagagatatcagcacagagatctaccaagcgggctcgacaccttgcaacggagtggagggcttcaactgttactttcctctgcagtcttatggcttccaacctacaaatggcgtcggatatcagccctacagagtggtggtgctttctttcgagctgctgcacgccccagctaccgtgtgtggtcctaagaagtcgacaaatctggtgaagaataagtgcgtgaattttaactttaacggcctgaccggcaccggcgtgctgaccgaatctaacaagaaattcctgcctttccagcagttcggtagagatatcgccgacaccaccgatgccgtgcgggaccctcaaacactggaaatcctggacataacaccttgcagcttcggcggagtcagcgtgatcacacctggcaccaacaccagcaaccaggtggccgtgctgtaccaggacgtgaactgcacagaagtgcctgtggcgatccacgctgatcagctgacacctacatggcgggtgtactcaacaggaagcaacgtgtttcagacacgggccggctgtctgatcggcgctgaacacgttaacaacagctacgagtgcgacatccccatcggcgccggcatctgtgccagctaccagactcagacaaatagccctaggagagcaagatccgtggccagccagagcatcatcgcctatacaatgagcctgggcgccgagaattctgtcgcctacagcaacaacagcatcgccatccccactaatttcaccatctccgtcaccacagaaatcctgcctgtgagcatgaccaagaccagcgtggattgcacaatgtacatttgcggcgacagcaccgagtgttccaacctgctgctgcagtacggcagcttctgcacccagctgaacagagcactgacaggcatcgccgtggagcaagacaagaacacccaggaggtgttcgcccaggtgaagcagatctacaagacccctcctatcaaagacttcggtggcttcaacttcagccagatcctgcctgatccgagcaagcctagcaaaagatcatttatcgaagacctgctgtttaacaaggtgaccctggccgacgccggattcatcaagcagtacggcgactgcctgggcgacatcgccgccagagatctgatctgtgcccagaagtttaatggcctgaccgtgctgccacctctgctgaccgacgagatgatcgcccaatataccagcgccctgctggctggaacaatcacaagcggctggaccttcggagccggagccgctcttcagattcctttcgccatgcagatggcctacagattcaacggcatcggcgtgacccagaacgtgctgtatgagaaccagaaactgatcgctaatcaatttaacagcgccatcggcaagattcaggactccctgagctcaacagcctctgccctgggcaagctgcaggatgtggtgaaccagaacgcccaggccctgaacacactggtgaaacagctgtcaagcaacttcggcgccatctcatccgtactgaacgacatcctgtctagactcgatccaccagaggccgaagtgcagatcgacagactgatcaccggccggctgcagagcctgcagacgtacgtgacccaacagctgatcagggccgccgagatccgggcctcggctaatttggccgccaccaaaatgagcgaatgcgtgctgggccagtctaagagggtcgacttctgtggcaagggctaccacctgatgagcttcccccagagcgctccccacggcgtggtgttcctgcacgtgacctacgttccagcccaggagaagaactttacaaccgcccctgccatctgccacgacggcaaggcccacttccctagagagggagtctttgtgagcaatggcacccactggttcgttacccagagaaacttctacgagccccagatcatcaccacagacaacaccttcgtgagcggaaactgtgacgtggtgatcggcatcgtgaacaacaccgtgtacgaccccctgcaacccgagctggacagcttcaaggaagagctggacaaatactttaagaaccacacctcacctgacgtggacctgggagatatcagcggcataaatgcctccgtggtgaacatccagaaggaaatcgatagactcaatgaggtggctaagaacctgaacgaaagcctgatcgacctccaagagctgggcaaatacgagcagtacatcaagtggccttggtacatttggctgggctttatcgccggcctcatcgctatcgtgatggtgaccatcatgctgtgctgcatgacctcctgctgcagctgcctgaagggctgttgcagctgcggcagctgctgcaagttcgacgaagatgattctgaaccagtgctgaaaggcgtgaaactgcactacaccagacagaaaagaatcgataagatcagcgacgtgtctacaatcgtgccatacatcggccctgccctgaatatccccaagaagcggaacaacttcaccgtcagcttctggctgagagtgcctaaggtgtccgccagccacctggagtga

SEQ ID NO: 50 - RNA, 4047 nt, Artificial Sequence
  F IX SP - SARS-CoV-2 S - TTTh
atgcaaagagttaacatgattatggctgaatctccaggtttgatcactatctgtttgttgggttacttgttatccgccgaatgtttcgtgttcctcgtcttgctacctttggtttcttctcaatgtgttaatttgactaccagaacccaattaccaccagcttacaccaattcttttaccagaggcgtgtactaccccgacaaggtgttccggagtagcgtgctgcacagcacgcaggacctgttcctgccatttttctctaatgtgacctggtttcacgccatccacgtgtccggcacaaacggcacaaagcggttcgacaaccccgtgctgccattcaacgatggcgtgtacttcgcctctacagaaaagtccaatatcattaggggctggatcttcggaacaacgctggactcaaagacccagagcctgctgatcgtcaataacgccacaaatgtggtcattaaagtgtgcgaattccagttctgcaacgaccccttcctgggcgtctactatcataagaacaacaagtcttggatggaaagcgagttccgggtgtacagcagcgctaacaactgcaccttcgagtacgtttcccaacctttcctgatggacctggaaggcaagcagggcaatttcaagaacctgagagaattcgtgttcaagaacatcgacggctacttcaagatctacagcaagcacacccccatcaacctggtacgagatctgccccagggcttctctgccctcgagcccctcgtggacctgcccattggaatcaacatcacgcggttccagaccctgctcgccctgcatagaagctacctcactcccggcgattctagcagcggctggacagccggcgctgccgcttactacgtgggctacctgcagcctagaacatttctactgaagtataacgagaacgggacaatcacagacgccgtggactgcgctctggatcctctgagcgaaaccaagtgcaccctgaaaagcttcaccgtcgagaagggaatctaccagacctccaacttccgggtgcagccaaccgagagcatcgtgagattccctaacatcactaacctgtgtccttttggagaagtgttcaacgccacccggttcgccagcgtttatgcctggaaccgcaagagaatctctaactgtgtggccgactacagcgtgctgtacaattctgccagcttcagcaccttcaagtgctacggcgtgagtcccaccaaactgaacgacctgtgcttcactaacgtgtacgccgatagctttgtgatcagaggagacgaggtgagacagattgctcctggccagaccggcaaaatcgccgattacaactacaagctacctgacgacttcaccggctgcgtgatcgcctggaattctaacaacctggactccaaggtgggcggcaactacaactacctgtacagactgtttcggaagtccaacctgaaaccattcgagagagatatcagcacagagatctaccaagcgggctcgacaccttgcaacggagtggagggcttcaactgttactttcctctgcagtcttatggcttccaacctacaaatggcgtcggatatcagccctacagagtggtggtgctttctttcgagctgctgcacgccccagctaccgtgtgtggtcctaagaagtcgacaaatctggtgaagaataagtgcgtgaattttaactttaacggcctgaccggcaccggcgtgctgaccgaatctaacaagaaattcctgcctttccagcagttcggtagagatatcgccgacaccaccgatgccgtgcgggaccctcaaacactggaaatcctggacataacaccttgcagcttcggcggagtcagcgtgatcacacctggcaccaacaccagcaaccaggtggccgtgctgtaccaggacgtgaactgcacagaagtgcctgtggcgatccacgctgatcagctgacacctacatggcgggtgtactcaacaggaagcaacgtgtttcagacacgggccggctgtctgatcggcgctgaacacgttaacaacagctacgagtgcgacatccccatcggcgccggcatctgtgccagctaccagactcagacaaatagccctaggagagcaagatccgtggccagccagagcatcatcgcctatacaatgagcctgggcgccgagaattctgtcgcctacagcaacaacagcatcgccatccccactaatttcaccatctccgtcaccacagaaatcctgcctgtgagcatgaccaagaccagcgtggattgcacaatgtacatttgcggcgacagcaccgagtgttccaacctgctgctgcagtacggcagcttctgcacccagctgaacagagcactgacaggcatcgccgtggagcaagacaagaacacccaggaggtgttcgcccaggtgaagcagatctacaagacccctcctatcaaagacttcggtggcttcaacttcagccagatcctgcctgatccgagcaagcctagcaaaagatcatttatcgaagacctgctgtttaacaaggtgaccctggccgacgccggattcatcaagcagtacggcgactgcctgggcgacatcgccgccagagatctgatctgtgcccagaagtttaatggcctgaccgtgctgccacctctgctgaccgacgagatgatcgcccaatataccagcgccctgctggctggaacaatcacaagcggctggaccttcggagccggagccgctcttcagattcctttcgccatgcagatggcctacagattcaacggcatcggcgtgacccagaacgtgctgtatgagaaccagaaactgatcgctaatcaatttaacagcgccatcggcaagattcaggactccctgagctcaacagcctctgccctgggcaagctgcaggatgtggtgaaccagaacgcccaggccctgaacacactggtgaaacagctgtcaagcaacttcggcgccatctcatccgtactgaacgacatcctgtctagactcgatccaccagaggccgaagtgcagatcgacagactgatcaccggccggctgcagagcctgcagacgtacgtgacccaacagctgatcagggccgccgagatccgggcctcggctaatttggccgccaccaaaatgagcgaatgcgtgctgggccagtctaagagggtcgacttctgtggcaagggctaccacctgatgagcttcccccagagcgctccccacggcgtggtgttcctgcacgtgacctacgttccagcccaggagaagaactttacaaccgcccctgccatctgccacgacggcaaggcccacttccctagagagggagtctttgtgagcaatggcacccactggttcgttacccagagaaacttctacgagccccagatcatcaccacagacaacaccttcgtgagcggaaactgtgacgtggtgatcggcatcgtgaacaacaccgtgtacgaccccctgcaacccgagctggacagcttcaaggaagagctggacaaatactttaagaaccacacctcacctgacgtggacctgggagatatcagcggcataaatgcctccgtggtgaacatccagaaggaaatcgatagactcaatgaggtggctaagaacctgaacgaaagcctgatcgacctccaagagctgggcaaatacgagcagtacatcaagtggccttggtacatttggctgggctttatcgccggcctcatcgctatcgtgatggtgaccatcatgctgtgctgcatgacctcctgctgcagctgcctgaagggctgttgcagctgcggcagctgctgcaagttcgacgaagatgattctgaaccagtgctgaaaggcgtgaaactgcactacaccagacagaaaagaatcgataagatcagcgacgtgtctacaatcgtgccatacatcggccctgccctgaatatccccaagaagcggaacaacttcaccgtcagcttctggctgagagtgcctaaggtgtccgccagccacctggagtga

SEQ ID NO: 51 - RNA, 4023 nt, Artificial Sequence
  MLP1 SP - SARS-CoV-2 S - TTTh
atggtatataaaactttatttgctttatgtattttaactgctggttggcgtgtacaatctttcgtgttcctcgtcttgctacctttggtttcttctcaatgtgttaatttgactaccagaacccaattaccaccagcttacaccaattcttttaccagaggcgtgtactaccccgacaaggtgttccggagtagcgtgctgcacagcacgcaggacctgttcctgccatttttctctaatgtgacctggtttcacgccatccacgtgtccggcacaaacggcacaaagcggttcgacaaccccgtgctgccattcaacgatggcgtgtacttcgcctctacagaaaagtccaatatcattaggggctggatcttcggaacaacgctggactcaaagacccagagcctgctgatcgtcaataacgccacaaatgtggtcattaaagtgtgcgaattccagttctgcaacgaccccttcctgggcgtctactatcataagaacaacaagtcttggatggaaagcgagttccgggtgtacagcagcgctaacaactgcaccttcgagtacgtttcccaacctttcctgatggacctggaaggcaagcagggcaatttcaagaacctgagagaattcgtgttcaagaacatcgacggctacttcaagatctacagcaagcacacccccatcaacctggtacgagatctgccccagggcttctctgccctcgagcccctcgtggacctgcccattggaatcaacatcacgcggttccagaccctgctcgccctgcatagaagctacctcactcccggcgattctagcagcggctggacagccggcgctgccgcttactacgtgggctacctgcagcctagaacatttctactgaagtataacgagaacgggacaatcacagacgccgtggactgcgctctggatcctctgagcgaaaccaagtgcaccctgaaaagcttcaccgtcgagaagggaatctaccagacctccaacttccgggtgcagccaaccgagagcatcgtgagattccctaacatcactaacctgtgtccttttggagaagtgttcaacgccacccggttcgccagcgtttatgcctggaaccgcaagagaatctctaactgtgtggccgactacagcgtgctgtacaattctgccagcttcagcaccttcaagtgctacggcgtgagtcccaccaaactgaacgacctgtgcttcactaacgtgtacgccgatagctttgtgatcagaggagacgaggtgagacagattgctcctggccagaccggcaaaatcgccgattacaactacaagctacctgacgacttcaccggctgcgtgatcgcctggaattctaacaacctggactccaaggtgggcggcaactacaactacctgtacagactgtttcggaagtccaacctgaaaccattcgagagagatatcagcacagagatctaccaagcgggctcgacaccttgcaacggagtggagggcttcaactgttactttcctctgcagtcttatggcttccaacctacaaatggcgtcggatatcagccctacagagtggtggtgctttctttcgagctgctgcacgccccagctaccgtgtgtggtcctaagaagtcgacaaatctggtgaagaataagtgcgtgaattttaactttaacggcctgaccggcaccggcgtgctgaccgaatctaacaagaaattcctgcctttccagcagttcggtagagatatcgccgacaccaccgatgccgtgcgggaccctcaaacactggaaatcctggacataacaccttgcagcttcggcggagtcagcgtgatcacacctggcaccaacaccagcaaccaggtggccgtgctgtaccaggacgtgaactgcacagaagtgcctgtggcgatccacgctgatcagctgacacctacatggcgggtgtactcaacaggaagcaacgtgtttcagacacgggccggctgtctgatcggcgctgaacacgttaacaacagctacgagtgcgacatccccatcggcgccggcatctgtgccagctaccagactcagacaaatagccctaggagagcaagatccgtggccagccagagcatcatcgcctatacaatgagcctgggcgccgagaattctgtcgcctacagcaacaacagcatcgccatccccactaatttcaccatctccgtcaccacagaaatcctgcctgtgagcatgaccaagaccagcgtggattgcacaatgtacatttgcggcgacagcaccgagtgttccaacctgctgctgcagtacggcagcttctgcacccagctgaacagagcactgacaggcatcgccgtggagcaagacaagaacacccaggaggtgttcgcccaggtgaagcagatctacaagacccctcctatcaaagacttcggtggcttcaacttcagccagatcctgcctgatccgagcaagcctagcaaaagatcatttatcgaagacctgctgtttaacaaggtgaccctggccgacgccggattcatcaagcagtacggcgactgcctgggcgacatcgccgccagagatctgatctgtgcccagaagtttaatggcctgaccgtgctgccacctctgctgaccgacgagatgatcgcccaatataccagcgccctgctggctggaacaatcacaagcggctggaccttcggagccggagccgctcttcagattcctttcgccatgcagatggcctacagattcaacggcatcggcgtgacccagaacgtgctgtatgagaaccagaaactgatcgctaatcaatttaacagcgccatcggcaagattcaggactccctgagctcaacagcctctgccctgggcaagctgcaggatgtggtgaaccagaacgcccaggccctgaacacactggtgaaacagctgtcaagcaacttcggcgccatctcatccgtactgaacgacatcctgtctagactcgatccaccagaggccgaagtgcagatcgacagactgatcaccggccggctgcagagcctgcagacgtacgtgacccaacagctgatcagggccgccgagatccgggcctcggctaatttggccgccaccaaaatgagcgaatgcgtgctgggccagtctaagagggtcgacttctgtggcaagggctaccacctgatgagcttcccccagagcgctccccacggcgtggtgttcctgcacgtgacctacgttccagcccaggagaagaactttacaaccgcccctgccatctgccacgacggcaaggcccacttccctagagagggagtctttgtgagcaatggcacccactggttcgttacccagagaaacttctacgagccccagatcatcaccacagacaacaccttcgtgagcggaaactgtgacgtggtgatcggcatcgtgaacaacaccgtgtacgaccccctgcaacccgagctggacagcttcaaggaagagctggacaaatactttaagaaccacacctcacctgacgtggacctgggagatatcagcggcataaatgcctccgtggtgaacatccagaaggaaatcgatagactcaatgaggtggctaagaacctgaacgaaagcctgatcgacctccaagagctgggcaaatacgagcagtacatcaagtggccttggtacatttggctgggctttatcgccggcctcatcgctatcgtgatggtgaccatcatgctgtgctgcatgacctcctgctgcagctgcctgaagggctgttgcagctgcggcagctgctgcaagttcgacgaagatgattctgaaccagtgctgaaaggcgtgaaactgcactacaccagacagaaaagaatcgataagatcagcgacgtgtctacaatcgtgccatacatcggccctgccctgaatatccccaagaagcggaacaacttcaccgtcagcttctggctgagagtgcctaaggtgtccgccagccacctggagtga

SEQ ID NO: 52 - RNA, 864 nt, Artificial Sequence
  albumin SP - SARS-CoV-2 M - TTTh
atgaagtgggtaacctttatttcccttctttttctctttagctcggcttattccgctgattccaacggtaccatcaccgttgaagaattgaagaagttgctggaacaatggaacttggtcattggttttttattcttgacttggatctgtttgttgcaattcgcttacgctaacagaaaccgtttcctctacattatcaagttgatcttcctatggttattgtggccagtcactttggcttgtttcgttttggccgcagtttacagaatcaactggattacaggtggtattgctattgctatggcctgtctggtgggcctgatgtggctgagctacttcatcgcctcttttagactgtttgccagaacccggagcatgtggtccttcaaccccgagacaaacatcctgctgaatgtgcccctgcacggcacaatcctgacaagacctctgcttgagagcgagctggtgatcggcgccgtgatcctgaggggccatctgcggattgccggacaccacctgggcagatgcgacatcaaggacctgcctaaggaaatcaccgtggctacaagccgcaccctgtcctactacaaactcggcgccagccaaagagtggccggcgacagcggcttcgccgcctatagcagataccggatcggcaactacaagctgaacaccgaccactctagcagctctgataatatcgccctgctggttcagagacagaaaagaatcgataagatcagcgacgtgtctacaatcgtgccatacatcggccctgccctgaatatccccaagaagcggaacaacttcaccgtcagcttctggctgagagtgcctaaggtgtccgccagccacctggagtga

SEQ ID NO: 53 - RNA, 864 nt, Artificial Sequence
  albumin SP - SARS-CoV-2 M - TTTh
atgaagtgggttactttcatctctttgttgtttttattctcctctgcttactccgctgattccaacggtaccatcaccgttgaagaattgaagaagttgctggaacaatggaacttggtcattggttttttattcttgacttggatctgtttgttgcaattcgcttacgctaacagaaaccgtttcctctacattatcaagttgatcttcctatggttattgtggccagtcactttggcttgtttcgttttggccgcagtttacagaatcaactggattacaggtggtattgctattgctatggcctgtctggtgggcctgatgtggctgagctacttcatcgcctcttttagactgtttgccagaacccggagcatgtggtccttcaaccccgagacaaacatcctgctgaatgtgcccctgcacggcacaatcctgacaagacctctgcttgagagcgagctggtgatcggcgccgtgatcctgaggggccatctgcggattgccggacaccacctgggcagatgcgacatcaaggacctgcctaaggaaatcaccgtggctacaagccgcaccctgtcctactacaaactcggcgccagccaaagagtggccggcgacagcggcttcgccgcctatagcagataccggatcggcaactacaagctgaacaccgaccactctagcagctctgataatatcgccctgctggttcagagacagaaaagaatcgataagatcagcgacgtgtctacaatcgtgccatacatcggccctgccctgaatatccccaagaagcggaacaacttcaccgtcagcttctggctgagagtgcctaaggtgtccgccagccacctggagtga

SEQ ID NO: 54 - RNA, 879 nt, Artificial Sequence
  IFN-r SP - SARS-CoV-2 M - TTTh
atgaaatatacaagttatatcttggcttttcagctctgcatcgttttgggttctcttggctgttactgcgctgattccaacggtaccatcaccgttgaagaattgaagaagttgctggaacaatggaacttggtcattggttttttattcttgacttggatctgtttgttgcaattcgcttacgctaacagaaaccgtttcctctacattatcaagttgatcttcctatggttattgtggccagtcactttggcttgtttcgttttggccgcagtttacagaatcaactggattacaggtggtattgctattgctatggcctgtctggtgggcctgatgtggctgagctacttcatcgcctcttttagactgtttgccagaacccggagcatgtggtccttcaaccccgagacaaacatcctgctgaatgtgcccctgcacggcacaatcctgacaagacctctgcttgagagcgagctggtgatcggcgccgtgatcctgaggggccatctgcggattgccggacaccacctgggcagatgcgacatcaaggacctgcctaaggaaatcaccgtggctacaagccgcaccctgtcctactacaaactcggcgccagccaaagagtggccggcgacagcggcttcgccgcctatagcagataccggatcggcaactacaagctgaacaccgaccactctagcagctctgataatatcgccctgctggttcagagacagaaaagaatcgataagatcagcgacgtgtctacaatcgtgccatacatcggccctgccctgaatatccccaagaagcggaacaacttcaccgtcagcttctggctgagagtgcctaaggtgtccgccagccacctggagtga

SEQ ID NO: 55 - RNA, 879 nt, Artificial Sequence
  IFN-r SP - SARS-CoV-2 M - TTTh
atgaagtacacttcttacattttggctttccaattgtgtatcgttttgggttccttaggttgttactgtgctgattccaacggtaccatcaccgttgaagaattgaagaagttgctggaacaatggaacttggtcattggttttttattcttgacttggatctgtttgttgcaattcgcttacgctaacagaaaccgtttcctctacattatcaagttgatcttcctatggttattgtggccagtcactttggcttgtttcgttttggccgcagtttacagaatcaactggattacaggtggtattgctattgctatggcctgtctggtgggcctgatgtggctgagctacttcatcgcctcttttagactgtttgccagaacccggagcatgtggtccttcaaccccgagacaaacatcctgctgaatgtgcccctgcacggcacaatcctgacaagacctctgcttgagagcgagctggtgatcggcgccgtgatcctgaggggccatctgcggattgccggacaccacctgggcagatgcgacatcaaggacctgcctaaggaaatcaccgtggctacaagccgcaccctgtcctactacaaactcggcgccagccaaagagtggccggcgacagcggcttcgccgcctatagcagataccggatcggcaactacaagctgaacaccgaccactctagcagctctgataatatcgccctgctggttcagagacagaaaagaatcgataagatcagcgacgtgtctacaatcgtgccatacatcggccctgccctgaatatccccaagaagcggaacaacttcaccgtcagcttctggctgagagtgcctaaggtgtccgccagccacctggagtga

SEQ ID NO: 56 - RNA, 894 nt, Artificial Sequence
  F IX SP - SARS-CoV-2 M - TTTh
atgcagcgcgtgaacatgatcatggcagaatcaccaggcctcatcaccatctgccttttaggatatctactcagtgctgaatgtgctgattccaacggtaccatcaccgttgaagaattgaagaagttgctggaacaatggaacttggtcattggttttttattcttgacttggatctgtttgttgcaattcgcttacgctaacagaaaccgtttcctctacattatcaagttgatcttcctatggttattgtggccagtcactttggcttgtttcgttttggccgcagtttacagaatcaactggattacaggtggtattgctattgctatggcctgtctggtgggcctgatgtggctgagctacttcatcgcctcttttagactgtttgccagaacccggagcatgtggtccttcaaccccgagacaaacatcctgctgaatgtgcccctgcacggcacaatcctgacaagacctctgcttgagagcgagctggtgatcggcgccgtgatcctgaggggccatctgcggattgccggacaccacctgggcagatgcgacatcaaggacctgcctaaggaaatcaccgtggctacaagccgcaccctgtcctactacaaactcggcgccagccaaagagtggccggcgacagcggcttcgccgcctatagcagataccggatcggcaactacaagctgaacaccgaccactctagcagctctgataatatcgccctgctggttcagagacagaaaagaatcgataagatcagcgacgtgtctacaatcgtgccatacatcggccctgccctgaatatccccaagaagcggaacaacttcaccgtcagcttctggctgagagtgcctaaggtgtccgccagccacctggagtga

SEQ ID NO: 57 - RNA, 894 nt, Artificial Sequence
  F IX SP - SARS-CoV-2 M - TTTh
atgcaaagagttaacatgattatggctgaatctccaggtttgatcactatctgtttgttgggttacttgttatccgccgaatgtgctgattccaacggtaccatcaccgttgaagaattgaagaagttgctggaacaatggaacttggtcattggttttttattcttgacttggatctgtttgttgcaattcgcttacgctaacagaaaccgtttcctctacattatcaagttgatcttcctatggttattgtggccagtcactttggcttgtttcgttttggccgcagtttacagaatcaactggattacaggtggtattgctattgctatggcctgtctggtgggcctgatgtggctgagctacttcatcgcctcttttagactgtttgccagaacccggagcatgtggtccttcaaccccgagacaaacatcctgctgaatgtgcccctgcacggcacaatcctgacaagacctctgcttgagagcgagctggtgatcggcgccgtgatcctgaggggccatctgcggattgccggacaccacctgggcagatgcgacatcaaggacctgcctaaggaaatcaccgtggctacaagccgcaccctgtcctactacaaactcggcgccagccaaagagtggccggcgacagcggcttcgccgcctatagcagataccggatcggcaactacaagctgaacaccgaccactctagcagctctgataatatcgccctgctggttcagagacagaaaagaatcgataagatcagcgacgtgtctacaatcgtgccatacatcggccctgccctgaatatccccaagaagcggaacaacttcaccgtcagcttctggctgagagtgcctaaggtgtccgccagccacctggagtga

SEQ ID NO: 58 - RNA, 870 nt, Artificial Sequence
  MLP1 SP - SARS-CoV-2 M - TTTh
atggtctacaagactctcttcgctctttgcatcttaactgcaggatggagggtacagagtgctgattccaacggtaccatcaccgttgaagaattgaagaagttgctggaacaatggaacttggtcattggttttttattcttgacttggatctgtttgttgcaattcgcttacgctaacagaaaccgtttcctctacattatcaagttgatcttcctatggttattgtggccagtcactttggcttgtttcgttttggccgcagtttacagaatcaactggattacaggtggtattgctattgctatggcctgtctggtgggcctgatgtggctgagctacttcatcgcctcttttagactgtttgccagaacccggagcatgtggtccttcaaccccgagacaaacatcctgctgaatgtgcccctgcacggcacaatcctgacaagacctctgcttgagagcgagctggtgatcggcgccgtgatcctgaggggccatctgcggattgccggacaccacctgggcagatgcgacatcaaggacctgcctaaggaaatcaccgtggctacaagccgcaccctgtcctactacaaactcggcgccagccaaagagtggccggcgacagcggcttcgccgcctatagcagataccggatcggcaactacaagctgaacaccgaccactctagcagctctgataatatcgccctgctggttcagagacagaaaagaatcgataagatcagcgacgtgtctacaatcgtgccatacatcggccctgccctgaatatccccaagaagcggaacaacttcaccgtcagcttctggctgagagtgcctaaggtgtccgccagccacctggagtga

SEQ ID NO: 59 - RNA, 870 nt, Artificial Sequence
  MLP1 SP - SARS-CoV-2 M - TTTh
atggtatataaaactttatttgctttatgtattttaactgctggttggcgtgtacaatctgctgattccaacggtaccatcaccgttgaagaattgaagaagttgctggaacaatggaacttggtcattggttttttattcttgacttggatctgtttgttgcaattcgcttacgctaacagaaaccgtttcctctacattatcaagttgatcttcctatggttattgtggccagtcactttggcttgtttcgttttggccgcagtttacagaatcaactggattacaggtggtattgctattgctatggcctgtctggtgggcctgatgtggctgagctacttcatcgcctcttttagactgtttgccagaacccggagcatgtggtccttcaaccccgagacaaacatcctgctgaatgtgcccctgcacggcacaatcctgacaagacctctgcttgagagcgagctggtgatcggcgccgtgatcctgaggggccatctgcggattgccggacaccacctgggcagatgcgacatcaaggacctgcctaaggaaatcaccgtggctacaagccgcaccctgtcctactacaaactcggcgccagccaaagagtggccggcgacagcggcttcgccgcctatagcagataccggatcggcaactacaagctgaacaccgaccactctagcagctctgataatatcgccctgctggttcagagacagaaaagaatcgataagatcagcgacgtgtctacaatcgtgccatacatcggccctgccctgaatatccccaagaagcggaacaacttcaccgtcagcttctggctgagagtgcctaaggtgtccgccagccacctggagtga